European Patent Application EP 4 600 267 A2, published August 13, 2025. Title: TARGETED LIGAND-PAYLOAD BASED DRUG DELIVERY FOR CELL THERAPY. Applicant: Purdue Research Foundation. Application EP. The sequence listing filed with the application follows.

SEQUENCE LISTING (22 sequences)

SEQ ID NO: 1 - protein, 367 aa, synthetic construct
  REGION 1..367: note = A synthetic amino acid sequence for mouse FKBP-FRa with linker peptide
MAHLMTVQLLLLVMWMAECAQSRAGVQVETISPGDGRTFPKRGQTCVVHYTGMLEDGKKFDSSRDRNKPFKFTLGKQEVIRGWEEGVAQMSVGQRAKLIISSDYAYGATGHPGIIPPHATLVFDVELLKLESGGGSTRARTELLNVCMDAKHHKEKPGPEDNLHDQCSPWKTNSCCSTNTSQEAHKDISYLYRFNWNHCGTMTSECKRHFIQDTCLYECSPNLGPWIQQVDQSWRKERILDVPLCKEDCQQWWEDCQSSFTCKSNWHKGWNWSSGHNECPVGASCHPFTFYFPTSAALCEEIWSHSYKLSNYSRGSGRCIQMWFDPAQGNPNEEVARFYAEAMSGAGFHGTWPLLCSLSLVLLWVIS

SEQ ID NO: 2 - protein, 369 aa, synthetic construct
  REGION 1..369: note = A synthetic amino acid sequence for human FKBP-FRa with linker peptide
MAQRMTTQLLLLLVWVAVVGEAQTGVQVETISPGDGRTFPKRGQTCVVHYTGMLEDGKKFDSSRDRNKPFKFMLGKQEVIRGWEEGVAQMSVGQRAKLTISPDYAYGATGHPGIIPPHATLVFDVELLKLESGGGSRIAWARTELLNVCMNAKHHKEKPGPEDKLHEQCRPWRKNACCSTNTSQEAHKDVSYLYRFNWNHCGEMAPACKRHFIQDTCLYECSPNLGPWIQQVDQSWRKERVLNVPLCKEDCEQWWEDCRTSYTCKSNWHKGWNWTSGFNKCAVGAACQPFHFYFPTPTVLCNEIWTHSYKVSNYSRGSGRCIQMWFDPAQGNPNEEVARFYAAAMSGAGPWAAWPFLLSLALMLLWLLS

SEQ ID NO: 3 - protein, 485 aa, synthetic construct
  REGION 1..485: note = A synthetic amino acid sequence for mouse antiCD19 CAR T construct
MGVPTQLLGLLLLWITDAICEQKLISEEDLDIQMTQSPASLSTSLGETVTIQCQASEDIYSGLAWYQQKPGKSPQLLIYGASDLQDGVPSRFSGSGSGTQYSLKITSMQTEDEGVYFCQQGLTYPRTFGGGTKLELKGGGGSGGGGSGGGGSEVQLQQSGAELVRPGTSVKLSCKVSGDTITFYYMHFVKQRPGQGLEWIGRIDPEDESTKYSEKFKNKATLTADTSSNTAYLKLSSLTSEDTATYFCIYGGYYFDYWGQGVMVTVSSIEFMYPPPYLDNERSNGTIIHIKEKHLCHTQSSPKLFWALVVVAGVLFCYGLLVTVALCVIWTNSRRNRGGQSDYMNMTPRRPGLTRKPYQPYAPARDFAAYRPRAKFSRSAETAANLQDPNQLYNELNLGRREEYDVLEKKRARDPEMGGKQQRRRNPQEGVYNALQKDKMAEAYSEIGTKGERRRGKGHDGLYQGLSTATKDTYDALHMQTLAPR

SEQ ID NO: 4 - protein, 496 aa, synthetic construct
  REGION 1..496: note = A synthetic amino acid sequence for human antiCD19 CAR T construct
MALPVTALLLPLALLLHAARPEQKLISEEDLDIQMTQTTSSLSASLGDRVTISCRASQDISKYLNWYQQKPDGTVKLLIYHTSRLHSGVPSRFSGSGSGTDYSLTISNLEQEDIATYFCQQGNTLPYTFGGGTKLEITGGGGSGGGGSGGGGSEVKLQESGPGLVAPSQSLSVTCTVSGVSLPDYGVSWIRQPPRKGLEWLGVIWGSETTYYNSALKSRLTIIKDNSKSQVFLKMNSLQTDDTAIYYCAKHYYYGGSYAMDYWGQGTSVTVSSAAAIEVMYPPPYLDNEKSNGTIIHVKGKHLCPSPLFPGPSKPFWVLVVVGGVLACYSLLVTVAFIIFWVRSKRSRLLHSDYMNMTPRRPGPTRKHYQPYAPPRDFAAYRSRVKFSRSADAPAYQQGQNQLYNELNLGRREEYDVLDKRRGRDPEMGGKPQRRKNPQEGLYNELQKDKMAEAYSEIGMKGERRRGKGHDGLYQGLSTATKDTYDALHMQALPPR

SEQ ID NO: 5 - DNA, 12182 bp, synthetic construct
  misc_feature 1..12182: note = A synthetic vector sequence for pWPI for human T cell transduction
  source 1..12182: mol_type = other DNA
ttggaagggctaattcactcccaaagaagacaagatatccttgatctgtggatctaccacacacaaggctacttccctgattagcagaactacacaccagggccaggggtcagatatccactgacctttggatggtgctacaagctagtaccagttgagccagataaggtagaagaggccaataaaggagagaacaccagcttgttacaccctgtgagcctgcatgggatggatgacccggagagagaagtgttagagtggaggtttgacagccgcctagcatttcatcacgtggcccgagagctgcatccggagtacttcaagaactgctgatatcgagcttgctacaagggactttccgctggggactttccagggaggcgtggcctgggcgggactggggagtggcgagccctcagatcctgcatataagcagctgctttttgcctgtactgggtctctctggttagaccagatctgagcctgggagctctctggctaactagggaacccactgcttaagcctcaataaagcttgccttgagtgcttcaagtagtgtgtgcccgtctgttgtgtgactctggtaactagagatccctcagacccttttagtcagtgtggaaaatctctagcagtggcgcccgaacagggacttgaaagcgaaagggaaaccagaggagctctctcgacgcaggactcggcttgctgaagcgcgcacggcaagaggcgaggggcggcgactggtgagtacgccaaaaattttgactagcggaggctagaaggagagagatgggtgcgagagcgtcagtattaagcgggggagaattagatcgcgatgggaaaaaattcggttaaggccagggggaaagaaaaaatataaattaaaacatatagtatgggcaagcagggagctagaacgattcgcagttaatcctggcctgttagaaacatcagaaggctgtagacaaatactgggacagctacaaccatcccttcagacaggatcagaagaacttagatcattatataatacagtagcaaccctctattgtgtgcatcaaaggatagagataaaagacaccaaggaagctttagacaagatagaggaagagcaaaacaaaagtaagaccaccgcacagcaagcggccgctgatcttcagacctggaggaggagatatgagggacaattggagaagtgaattatataaatataaagtagtaaaaattgaaccattaggagtagcacccaccaaggcaaagagaagagtggtgcagagagaaaaaagagcagtgggaataggagctttgttccttgggttcttgggagcagcaggaagcactatgggcgcagcgtcaatgacgctgacggtacaggccagacaattattgtctggtatagtgcagcagcagaacaatttgctgagggctattgaggcgcaacagcatctgttgcaactcacagtctggggcatcaagcagctccaggcaagaatcctggctgtggaaagatacctaaaggatcaacagctcctggggatttggggttgctctggaaaactcatttgcaccactgctgtgccttggaatgctagttggagtaataaatctctggaacagatttggaatcacacgacctggatggagtgggacagagaaattaacaattacacaagcttaatacactccttaattgaagaatcgcaaaaccagcaagaaaagaatgaacaagaattattggaattagataaatgggcaagtttgtggaattggtttaacataacaaattggctgtggtatataaaattattcataatgatagtaggaggcttggtaggtttaagaatagtttttgctgtactttctatagtgaatagagttaggcagggatattcaccattatcgtttcagacccacctcccaaccccgaggggacccgacaggcccgaaggaatagaagaagaaggtggagagagagacagagacagatccattcgattagtgaacggatctcgacggtatcgatgtcgacgataagctttgcaaagatggataaagttttaaacagagaggaatctttgcagctaatggaccttctaggtcttgaaaggagtgggaattggctccggtgcccgtcagtgggcagagcgcacatcgcccacagtccccgagaagttggggggaggggtcggcaattgaaccggtgcctagagaaggtggcgcggggtaaactgggaaagtgatgtcgtgtactggctccgcctttttcccgagggtgggggagaaccgtatataagtgcagtagtcgccgtgaacgttctttttcgcaacgggtttgccgccagaacacaggtaagtgccgtgtgtggttcccgcgggcctggcctctttacgggttatggcccttgcgtgccttgaattacttccactggctgcagtacgtgattcttgatcccgagcttcgggttggaagtgggtgggagagttcgaggccttgcgcttaaggagccccttcgcctcgtgcttgagttgaggcctggcctgggcgctggggccgccgcgtgcgaatctggtggcaccttcgcgcctgtctcgctgctttcgataagtctctagccatttaaaatttttgatgacctgctgcgacgctttttttctggcaagatagtcttgtaaatgcgggccaagatctgcacactggtatttcggtttttggggccgcgggcggcgacggggcccgtgcgtcccagcgcacatgttcggcgaggcggggcctgcgagcgcggccaccgagaatcggacgggggtagtctcaagctggccggcctgctctggtgcctggcctcgcgccgccgtgtatcgccccgccctgggcggcaaggctggcccggtcggcaccagttgcgtgagcggaaagatggccgcttcccggccctgctgcagggagctcaaaatggaggacgcggcgctcgggagagcgggcgggtgagtcacccacacaaaggaaaagggcctttccgtcctcagccgtcgcttcatgtgactccacggagtaccgggcgccgtccaggcacctcgattagttctcgagcttttggagtacgtcgtctttaggttggggggaggggttttatgcgatggagtttccccacactgagtgggtggagactgaagttaggccagcttggcacttgatgtaattctccttggaatttgccctttttgagtttggatcttggttcattctcaagcctcagacagtggttcaaagtttttttcttccatttcaggtgtcgtgaggaatttcgacatttaaatttaattaatctcgacggtatcggttaacttttaaaagaaaaggggggattggggggtacagtgcaggggaaagaatagtagacataatagcaacagacatacaaactaaagaattacaaaaacaaattacaaaaattcaaaattttatcgatcacgagactagcctcgaggtttatggctcacctgatgactgtgcagttgttgctcctggtgatgtggatggccgaatgtgctcagtccagagctggagtgcaggtggagaccatctctcctggagacgggcgcaccttcccaaagcgcggccagacctgcgtggtgcactacacggggatgcttgaagatggaaagaaatttgattcctctcgggacagaaacaagccttttaagtttacactaggcaagcaggaggtgatccgaggctgggaggaaggggtagcccagatgagtgtgggtcagagagccaaactgataatctcctcagactatgcctatggagccaccgggcacccaggcatcatcccaccacatgccactcttgtttttgatgtggagcttctaaaactggaaagcggcggcggcagcactcgggccaggactgaacttctcaatgtctgcatggatgccaaacaccacaaagaaaaaccgggccctgaggacaatttacacgaccagtgcagcccctggaagacgaattcctgctgttccacgaacacaagccaggaagcacataaggacatttcctacctgtaccggttcaactggaaccactgcggaactatgacatcggaatgcaaacggcactttatccaagacacctgcctctatgagtgttccccgaacttgggaccctggatccagcaggtggaccagagctggcgcaaagagcggatccttgatgttcccctgtgcaaagaggactgtcagcagtggtgggaggactgccagagctcttttacctgcaagagcaattggcacaagggatggaactggtcctcggggcataacgagtgtcctgtgggagcctcctgccatcccttcaccttctacttccccacatctgctgctctgtgtgaggaaatctggagtcactcctacaagctcagcaactacagtcgagggagcggccgctgcattcagatgtggttcgacccagcccagggcaaccccaacgaggaagtggcgaggttctatgccgaggccatgagtggagctgggtttcatgggacctggccactcttgtgcagcctgtccttagtgctgctctgggtgatcagctgaaaactacgggctgcaggaattccgcccccccccccctaacgttactggccgaagccgcttggaataaggccggtgtgcgtttgtctatatgttattttccaccatattgccgtcttttggcaatgtgagggcccggaaacctggccctgtcttcttgacgagcattcctaggggtctttcccctctcgccaaaggaatgcaaggtctgttgaatgtcgtgaaggaagcagttcctctggaagcttcttgaagacaaacaacgtctgtagcgaccctttgcaggcagcggaaccccccacctggcgacaggtgcctctgcggccaaaagccacgtgtataagatacacctgcaaaggcggcacaaccccagtgccacgttgtgagttggatagttgtggaaagagtcaaatggctctcctcaagcgtattcaacaaggggctgaaggatgcccagaaggtaccccattgtatgggatctgatctggggcctcggtgcacatgctttacatgtgtttagtcgaggttaaaaaacgtctaggccccccgaaccacggggacgtggttttcctttgaaaaacacgatgataataccatggtgagcaagggcgaggagctgttcaccggggtggtgcccatcctggtcgagctggacggcgacgtaaacggccacaagttcagcgtgtccggcgagggcgagggcgatgccacctacggcaagctgaccctgaagttcatctgcaccaccggcaagctgcccgtgccctggcccaccctcgtgaccaccctgacctacggcgtgcagtgcttcagccgctaccccgaccacatgaagcagcacgacttcttcaagtccgccatgcccgaaggctacgtccaggagcgcaccatcttcttcaaggacgacggcaactacaagacccgcgccgaggtgaagttcgagggcgacaccctggtgaaccgcatcgagctgaagggcatcgacttcaaggaggacggcaacatcctggggcacaagctggagtacaactacaacagccacaacgtctatatcatggccgacaagcagaagaacggcatcaaggtgaacttcaagatccgccacaacatcgaggacggcagcgtgcagctcgccgaccactaccagcagaacacccccatcggcgacggccccgtgctgctgcccgacaaccactacctgagcacccagtccgccctgagcaaagaccccaacgagaagcgcgatcacatggtcctgctggagttcgtgaccgccgccgggatcactctcggcatggacgagctgtacaagtccggactcagatctcgactagctagtagctagctagctagtcgagctcaagcttcgaattcgatatcaagcttatcgcgataccgtcgacctcgagggaattccgataatcaacctctggattacaaaatttgtgaaagattgactggtattcttaactatgttgctccttttacgctatgtggatacgctgctttaatgcctttgtatcatgctattgcttcccgtatggctttcattttctcctccttgtataaatcctggttgctgtctctttatgaggagttgtggcccgttgtcaggcaacgtggcgtggtgtgcactgtgtttgctgacgcaacccccactggttggggcattgccaccacctgtcagctcctttccgggactttcgctttccccctccctattgccacggcggaactcatcgccgcctgccttgcccgctgctggacaggggctcggctgttgggcactgacaattccgtggtgttgtcggggaagctgacgtcctttccatggctgctcgcctgtgttgccacctggattctgcgcgggacgtccttctgctacgtcccttcggccctcaatccagcggaccttccttcccgcggcctgctgccggctctgcggcctcttccgcgtcttcgccttcgccctcagacgagtcggatctccctttgggccgcctccccgcatcgggaattcgagctcggtacctttaagaccaatgacttacaaggcagctgtagatcttagccactttttaaaagaaaaggggggactggaagggctaattcactcccaacgaagacaagatgggatcaattcaccatgggaataacttcgtatagcatacattatacgaagttatgctgctttttgcttgtactgggtctctctggttagaccagatctgagcctgggagctctctggctaactagggaacccactgcttaagcctcaataaagcttgccttgagtgcttcaagtagtgtgtgcccgtctgttgtgtgactctggtaactagagatccctcagacccttttagtcagtgtggaaaatctctagcagcatctagaattaattccgtgtattctatagtgtcacctaaatcgtatgtgtatgatacataaggttatgtattaattgtagccgcgttctaacgacaatatgtacaagcctaattgtgtagcatctggcttactgaagcagaccctatcatctctctcgtaaactgccgtcagagtcggtttggttggacgaaccttctgagtttctggtaacgccgtcccgcacccggaaatggtcagcgaaccaatcagcagggtcatcgctagccagatcctctacgccggacgcatcgtggccggcatcaccggcgccacaggtgcggttgctggcgcctatatcgccgacatcaccgatggggaagatcgggctcgccacttcgggctcatgagcgcttgtttcggcgtgggtatggtggcaggccccgtggccgggggactgttgggcgccatctccttgcatgcaccattccttgcggcggcggtgctcaacggcctcaacctactactgggctgcttcctaatgcaggagtcgcataagggagagcgtcgaatggtgcactctcagtacaatctgctctgatgccgcatagttaagccagccccgacacccgccaacacccgctgacgcgccctgacgggcttgtctgctcccggcatccgcttacagacaagctgtgaccgtctccgggagctgcatgtgtcagaggttttcaccgtcatcaccgaaacgcgcgagacgaaagggcctcgtgatacgcctatttttataggttaatgtcatgataataatggtttcttagacgtcaggtggcacttttcggggaaatgtgcgcggaacccctatttgtttatttttctaaatacattcaaatatgtatccgctcatgagacaataaccctgataaatgcttcaataatattgaaaaaggaagagtatgagtattcaacatttccgtgtcgcccttattcccttttttgcggcattttgccttcctgtttttgctcacccagaaacgctggtgaaagtaaaagatgctgaagatcagttgggtgcacgagtgggttacatcgaactggatctcaacagcggtaagatccttgagagttttcgccccgaagaacgttttccaatgatgagcacttttaaagttctgctatgtggcgcggtattatcccgtattgacgccgggcaagagcaactcggtcgccgcatacactattctcagaatgacttggttgagtactcaccagtcacagaaaagcatcttacggatggcatgacagtaagagaattatgcagtgctgccataaccatgagtgataacactgcggccaacttacttctgacaacgatcggaggaccgaaggagctaaccgcttttttgcacaacatgggggatcatgtaactcgccttgatcgttgggaaccggagctgaatgaagccataccaaacgacgagcgtgacaccacgatgcctgtagcaatggcaacaacgttgcgcaaactattaactggcgaactacttactctagcttcccggcaacaattaatagactggatggaggcggataaagttgcaggaccacttctgcgctcggcccttccggctggctggtttattgctgataaatctggagccggtgagcgtgggtctcgcggtatcattgcagcactggggccagatggtaagccctcccgtatcgtagttatctacacgacggggagtcaggcaactatggatgaacgaaatagacagatcgctgagataggtgcctcactgattaagcattggtaactgtcagaccaagtttactcatatatactttagattgatttaaaacttcatttttaatttaaaaggatctaggtgaagatcctttttgataatctcatgaccaaaatcccttaacgtgagttttcgttccactgagcgtcagaccccgtagaaaagatcaaaggatcttcttgagatcctttttttctgcgcgtaatctgctgcttgcaaacaaaaaaaccaccgctaccagcggtggtttgtttgccggatcaagagctaccaactctttttccgaaggtaactggcttcagcagagcgcagataccaaatactgtccttctagtgtagccgtagttaggccaccacttcaagaactctgtagcaccgcctacatacctcgctctgctaatcctgttaccagtggctgctgccagtggcgataagtcgtgtcttaccgggttggactcaagacgatagttaccggataaggcgcagcggtcgggctgaacggggggttcgtgcacacagcccagcttggagcgaacgacctacaccgaactgagatacctacagcgtgagcattgagaaagcgccacgcttcccgaagggagaaaggcggacaggtatccggtaagcggcagggtcggaacaggagagcgcacgagggagcttccagggggaaacgcctggtatctttatagtcctgtcgggtttcgccacctctgacttgagcgtcgatttttgtgatgctcgtcaggggggcggagcctatggaaaaacgccagcaacgcggcctttttacggttcctggccttttgctggccttttgctcacatgttctttcctgcgttatcccctgattctgtggataaccgtattaccgcctttgagtgagctgataccgctcgccgcagccgaacgaccgagcgcagcgagtcagtgagcgaggaagcggaagagcgcccaatacgcaaaccgcctctccccgcgcgttggccgattcattaatgcagctgtggaatgtgtgtcagttagggtgtggaaagtccccaggctccccagcaggcagaagtatgcaaagcatgcatctcaattagtcagcaaccaggtgtggaaagtccccaggctccccagcaggcagaagtatgcaaagcatgcatctcaattagtcagcaaccatagtcccgcccctaactccgcccatcccgcccctaactccgcccagttccgcccattctccgccccatggctgactaattttttttatttatgcagaggccgaggccgcctcggcctctgagctattccagaagtagtgaggaggcttttttggaggcctaggcttttgcaaaaagcttggacacaagacaggcttgcgagatatgtttgagaataccactttatcccgcgtcagggagaggcagtgcgtaaaaagacgcggactcatgtgaaatactggtttttagtgcgccagatctctataatctcgcgcaacctattttcccctcgaacactttttaagccgtagataaacaggctgggacacttcacatgagcgaaaaatacatcgtcacctgggacatgttgcagatccatgcacgtaaactcgcaagccgactgatgccttctgaacaatggaaaggcattattgccgtaagccgtggcggtctgtaccgggtgcgttactggcgcgtgaactgggtattcgtcatgtcgataccgtttgtatttccagctacgatcacgacaaccagcgcgagcttaaagtgctgaaacgcgcagaaggcgatggcgaaggcttcatcgttattgatgacctggtggataccggtggtactgcggttgcgattcgtgaaatgtatccaaaagcgcactttgtcaccatcttcgcaaaaccggctggtcgtccgctggttgatgactatgttgttgatatcccgcaagatacctggattgaacagccgtgggatatgggcgtcgtattcgtcccgccaatctccggtcgctaatcttttcaacgcctggcactgccgggcgttgttctttttaacttcaggcgggttacaatagtttccagtaagtattctggaggctgcatccatgacacaggcaaacctgagcgaaaccctgttcaaaccccgctttaaacatcctgaaacctcgacgctagtccgccgctttaatcacggcgcacaaccgcctgtgcagtcggcccttgatggtaaaaccatccctcactggtatcgcatgattaaccgtctgatgtggatctggcgcggcattgacccacgcgaaatcctcgacgtccaggcacgtattgtgatgagcgatgccgaacgtaccgacgatgatttatacgatacggtgattggctaccgtggcggcaactggatttatgagtgggccccggatctttgtgaaggaaccttacttctgtggtgtgacataattggacaaactacctacagagatttaaagctctaaggtaaatataaaatttttaagtgtataatgtgttaaactactgattctaattgtttgtgtattttagattccaacctatggaactgatgaatgggagcagtggtggaatgcctttaatgaggaaaacctgttttgctcagaagaaatgccatctagtgatgatgaggctactgctgactctcaacattctactcctccaaaaaagaagagaaaggtagaagaccccaaggactttccttcagaattgctaagttttttgagtcatgctgtgtttagtaatagaactcttgcttgctttgctatttacaccacaaaggaaaaagctgcactgctatacaagaaaattatggaaaaatattctgtaacctttataagtaggcataacagttataatcataacatactgttttttcttactccacacaggcatagagtgtctgctattaataactatgctcaaaaattgtgtacctttagctttttaatttgtaaaggggttaataaggaatatttgatgtatagtgccttgactagagatcataatcagccataccacatttgtagaggttttacttgctttaaaaaacctcccacacctccccctgaacctgaaacataaaatgaatgcaattgttgttgttaacttgtttattgcagcttataatggttacaaataaagcaatagcatcacaaatttcacaaataaagcatttttttcactgcattctagttgtggtttgtccaaactcatcaatgtatcttatcatgtctggatcaactggataactcaagctaaccaaaatcatcccaaacttcccaccccataccctattaccactgccaattacctagtggtttcatttactctaaacctgtgattcctctgaattattttcattttaaagaaattgtatttgttaaatatgtactacaaacttagtag

SEQ ID NO: 6 - DNA, 6939 bp, synthetic construct
  misc_feature 1..6939: note = A synthetic pMP71 gb NotIEcoRI mouse antiCD19 for mouse T cell transduction
  source 1..6939: mol_type = other DNA
tcaaggttaggaacagagagacaggagaatatgggccaaacaggatatctgtggtaagcagttcctgccccggctcagggccaagaacagttggaacagcagaatatgggccaaacaggatatctgtggtaagcagttcctgccccggctcagggccaagaacagatggtccccagatgcggtcccgccctcagcagtttctagagaaccatcagatgtttccagggtgccccaaggacctgaaatgaccctgtgccttatttgaactaaccaatcagttcgcttctcgcttctgttcgcgcgcttctgctccccgagctcaataaaagagcccacaacccctcactcggcgcgccagtcctccgattgactgcgtcgcccgggtacccgtattcccaataaagcctcttgctgtttgcatccgaatcgtggactcgctgatccttgggagggtctcctcagattgattgactgcccacctcgggggtctttcatttggaggttccaccgagatttggagacccctgcccagggaccaccgacccccccgccgggaggtaagctggccagcggtcgtttcgtgtctgtctctgtctttgggcgtgtttgtgccggcatctaatgtttgcgcctgcgtctgtactagttggctaactagatctgtatctggcggtcccgcggaagaactgacgagttcgtattcccggccgcagcccctgggagacgtcccagcggcctcgggggcccgttttgtggcccattctgtatcagttaacctacccgagtcggactttttggagctccgccactgtccgaggggtacgtggctttgttgggggacgagagacagagacacttcccgcccccgtctgaatttttgctttcggttttacgccgaaaccgcgccgcgcgtcttgtctgctgcagcatcgttctgtgttgtctctgtctgactgtgtttctgtatttgtctgaaaattagctcgacaaagttaagtaatagtccctctctccaagctcacttacaggcatgggggttcccacccagctgttggggttgctgctcctctggatcactgatgccatctgcgaacagaagctcatttctgaagaagatctggacatacagatgacccagagtcctgccagcttgtccacatccctcggagagaccgtgacaattcaatgccaggcctctgaggacatatattctggattggcttggtaccagcaaaagccaggtaaaagtcctcagttgttgatatacggcgcttctgatttgcaagacggggtgccctcacgatttagcgggtctggaagtggcactcagtacagtctgaagattacttcaatgcaaacagaagacgagggtgtgtatttttgccaacaggggctgacctacccaaggacattcgggggcggtacaaagcttgaacttaagggcggcggtgggtctggaggtggtggatctggcggagggggaagtgaggtacagctgcaacagtccggcgccgaactcgttcgccctggaacctcagtcaaattgtcatgcaaggtgagtggcgacacaataaccttttactatatgcacttcgttaaacagaggccaggtcaaggtctggaatggataggcagaattgatccagaagatgagtccaccaaatactcagaaaagttcaaaaacaaagccactcttactgccgacacctcaagcaacacagcatatcttaagctcagttcacttaccagcgaagacaccgccacctatttttgtatttatggtggctattactttgactactgggggcaaggtgttatggtaacagtttcttccattgaattcatgtatccacccccctatttggataatgaacgatctaatgggactataatacatatcaaggaaaagcatctgtgtcatacccaaagttcccctaagcttttctgggccctcgtcgttgtggcaggagtgcttttttgctatggattgttggttactgtggctctctgcgtcatttggacaaatagtaggaggaatcgggggggacaatctgattacatgaacatgacaccacggaggccaggccttaccagaaagccctaccaaccttatgcaccagcacgagacttcgccgcatacaggccaagggctaagttttcccgcagcgccgaaaccgcagccaacctccaagatcctaatcagctctataacgaattgaatcttggccgcagagaggagtacgacgtacttgagaaaaagagagctagggaccctgaaatgggtgggaagcaacagcgaagaaggaacccacaggaaggggtgtataatgcccttcaaaaggataaaatggcagaggcatacagtgaaatcggaaccaagggggagagacgcagagggaaaggccatgacggcctttatcagggtttgtcaactgctactaaagacacttatgatgccttgcatatgcaaactctcgcacccagatgacgagcatcttaccgccatttattcccatatttgttctgtttttcttgatttgggtatacatttaaatgttaataaaacaaaatggtggggcaatcatttacattttatgggatatgtaattactagttcaggtgtattgccacaagacaaacatgttaagaaactttcccgttatttacgctctgttcctgttaatcaacctctggattacaaaatttgtgaaagattgactgatattcttaactatgttgctccttttacgctgtgtggatatgctgctttaatgcctctgtatcatgctattgcttcccgtacggctttcgttttctcctccttgtataaatcctggttgctgtctctttatgaggagttgtggcccgttgtccgtcaacgtggcgtggtgtgctctgtgtttgctgacgcaacccccactggctggggcattgccaccacctgtcaactcctttctgggactttcgctttccccctcccgatcgccacggcagaactcatcgccgcctgccttgcccgctgctggacaggggctaggttgctgggcactgataattccgtggtgttgtcggggaagctgacgtcctttccatggctgctcgcctgtgttgccaactggatcctgcgcgggacgtccttctgctacgtcccttcggctctcaatccagcggacctcccttcccgaggccttctgccggttctgcggcctctcccgcgtcttcgctttcggcctccgacgagtcggatctccctttgggccgcctccccgcctgtttcgcctcggcgtccggtccgtgttgcttggtcgtcacctgtgcagaattgcgaaccatggattccaccgtgaactttgtctcctggcatgcaaatcgtcaacttggcatgccaagaattaattcggatccaagcttaggcctgctcgctttcttgctgtcccatttctattaaaggttcctttgttccctaagtccaactactaaactgggggatattatgaagggccttgagcatctggattctgcctagcgctaagcttcctaacacgagccatagatagaataaaagattttatttagtctccagaaaaaggggggaatgaaagaccccacctgtaggtttggcaagctagcttaagtaagccattttgcaaggcatggaaaaatacataactgagaatagagaagttcagatcaaggttaggaacagagagacaggagaatatgggccaaacaggatatctgtggtaagcagttcctgccccggctcagggccaagaacagttggaacagcagaatatgggccaaacaggatatctgtggtaagcagttcctgccccggctcagggccaagaacagatggtccccagatgcggtcccgccctcagcagtttctagagaaccatcagatgtttccagggtgccccaaggacctgaaatgaccctgtgccttatttgaactaaccaatcagttcgcttctcgcttctgttcgcgcgcttctgctccccgagctcaataaaagagcccacaacccctcactcggcgcgccagtcctccgatagactgcgtcgcccggggtacccgtattcccaataaagcctcttgctgtttgcatccgaatcgtggactcgctgatccttgggagggtctcctcagattgattgactgcccacctcgggggtctttcattctcgagagctttggcgtaatcatggtcatagctgtttcctgtgtgaaattgttatccgctcacaattccacacaacatacgagccggaagcataaagtgtaaagcctggggtgcctaatgagtgagctaactcacattaattgcgttgcgctcactgcccgctttccagtcgggaaacctgtcgtgccagctgcattaatgaatcggccaacgcgcggggagaggcggtttgcgtattgggcgctcttccgcttcctcgctcactgactcgctgcgctcggtcgttcggctgcggcgagcggtatcagctcactcaaaggcggtaatacggttatccacagaatcaggggataacgcaggaaagaacatgtgagcaaaaggccagcaaaaggccaggaaccgtaaaaaggccgcgttgctggcgtttttccataggctccgcccccctgacgagcatcacaaaaatcgacgctcaagtcagaggtggcgaaacccgacaggactataaagataccaggcgtttccccctggaagctccctcgtgcgctctcctgttccgaccctgccgcttaccggatacctgtccgcctttctcccttcgggaagcgtggcgctttctcaatgctcacgctgtaggtatctcagttcggtgtaggtcgttcgctccaagctgggctgtgtgcacgaaccccccgttcagcccgaccgctgcgccttatccggtaactatcgtcttgagtccaacccggtaagacacgacttatcgccactggcagcagccactggtaacaggattagcagagcgaggtatgtaggcggtgctacagagttcttgaagtggtggcctaactacggctacactagaaggacagtatttggtatctgcgctctgctgaagccagttaccttcggaaaaagagttggtagctcttgatccggcaaacaaaccaccgctggtagcggtggtttttttgtttgcaagcagcagattacgcgcagaaaaaaaggatctcaagaagatcctttgatcttttctacggggtctgacgctcagtggaacgaaaactcacgttaagggattttggtcatgagattatcaaaaaggatcttcacctagatccttttaaattaaaaatgaagttttaaatcaatctaaagtatatatgagtaaacttggtctgacagttaccaatgcttaatcagtgaggcacctatctcagcgatctgtctatttcgttcatccatagttgcctgactccccgtcgtgtagataactacgatacgggagggcttaccatctggccccagtgctgcaatgataccgcgagacccacgctcaccggctccagatttatcagcaataaaccagccagccggaagggccgagcgcagaagtggtcctgcaactttatccgcctccatccagtctattaattgttgccgggaagctagagtaagtagttcgccagttaatagtttgcgcaacgttgttgccattgctgctggcatcgtggtgtcacgctcgtcgtttggtatggcttcattcagctccggttcccaacgatcaaggcgagttacatgatcccccatgttgtgcaaaaaagcggttagctccttcggtcctccgatcgttgtcagaagtaagttggccgcagtgttatcactcatggttatggcagcactgcataattctcttactgtcatgccatccgtaagatgcttttctgtgactggtgagtactcaaccaagtcattctgagaatagtgtatgcggcgaccgagttgctcttgcccggcgtcaatacgggataataccgcgccacatagcagaactttaaaagtgctcatcattggaaaacgttcttcggggcgaaaactctcaaggatcttaccgctgttgagatccagttcgatgtaacccactcgtgcacccaactgatcttcagcatcttttactttcaccagcgtttctgggtgagcaaaaacaggaaggcaaaatgccgcaaaaaagggaataagggcgacacggaaatgttgaatactcatactcttcctttttcaatattattgaagcatttatcagggttattgtctcatgagcggatacatatttgaatgtatttagaaaaataaacaaataggggttccgcgcacatttccccgaaaagtgccacctgacgtctaagaaaccattattatcatgacattaacctataaaaataggcgtatcacgaggccctttcgtcttcaagctgcctcgcgcgtttcggtgatgacggtgaaaacctctgacacatgcagctcccggagacggtcacagcttgtctgtaagcggatgccgggagcagacaagcccgtcagggcgcgtcagcgggtgttggcgggtgtcggggcgcagccatgacccagtcacgtagcgatagttactatgcggcatcagagcagattgtactgagagtgcaccatatgcggtgtgaaataccgcacagatgcgtaaggagaaaataccgcatcaggcgccattcgccattcaggctgcgcaactgttgggaagggcgatcggtgcgggcctcttcgctattacgccagctggcgaaagggggatgtgctgcaaggcgattaagttgggtaacgccagggttttcccagtcacgacgttgtaaaacgacggccagtgaattagtactctagcttaagtaagccattttgcaaggcatggaaaaatacataactgagaatagagaagttcaga

SEQ ID NO: 7 - DNA, 12188 bp, synthetic construct
  misc_feature 1..12188: note = A synthetic pWPI-FRa 1-24 FKBP FRa
  source 1..12188: mol_type = other DNA
ttggaagggctaattcactcccaaagaagacaagatatccttgatctgtggatctaccacacacaaggctacttccctgattagcagaactacacaccagggccaggggtcagatatccactgacctttggatggtgctacaagctagtaccagttgagccagataaggtagaagaggccaataaaggagagaacaccagcttgttacaccctgtgagcctgcatgggatggatgacccggagagagaagtgttagagtggaggtttgacagccgcctagcatttcatcacgtggcccgagagctgcatccggagtacttcaagaactgctgatatcgagcttgctacaagggactttccgctggggactttccagggaggcgtggcctgggcgggactggggagtggcgagccctcagatcctgcatataagcagctgctttttgcctgtactgggtctctctggttagaccagatctgagcctgggagctctctggctaactagggaacccactgcttaagcctcaataaagcttgccttgagtgcttcaagtagtgtgtgcccgtctgttgtgtgactctggtaactagagatccctcagacccttttagtcagtgtggaaaatctctagcagtggcgcccgaacagggacttgaaagcgaaagggaaaccagaggagctctctcgacgcaggactcggcttgctgaagcgcgcacggcaagaggcgaggggcggcgactggtgagtacgccaaaaattttgactagcggaggctagaaggagagagatgggtgcgagagcgtcagtattaagcgggggagaattagatcgcgatgggaaaaaattcggttaaggccagggggaaagaaaaaatataaattaaaacatatagtatgggcaagcagggagctagaacgattcgcagttaatcctggcctgttagaaacatcagaaggctgtagacaaatactgggacagctacaaccatcccttcagacaggatcagaagaacttagatcattatataatacagtagcaaccctctattgtgtgcatcaaaggatagagataaaagacaccaaggaagctttagacaagatagaggaagagcaaaacaaaagtaagaccaccgcacagcaagcggccgctgatcttcagacctggaggaggagatatgagggacaattggagaagtgaattatataaatataaagtagtaaaaattgaaccattaggagtagcacccaccaaggcaaagagaagagtggtgcagagagaaaaaagagcagtgggaataggagctttgttccttgggttcttgggagcagcaggaagcactatgggcgcagcgtcaatgacgctgacggtacaggccagacaattattgtctggtatagtgcagcagcagaacaatttgctgagggctattgaggcgcaacagcatctgttgcaactcacagtctggggcatcaagcagctccaggcaagaatcctggctgtggaaagatacctaaaggatcaacagctcctggggatttggggttgctctggaaaactcatttgcaccactgctgtgccttggaatgctagttggagtaataaatctctggaacagatttggaatcacacgacctggatggagtgggacagagaaattaacaattacacaagcttaatacactccttaattgaagaatcgcaaaaccagcaagaaaagaatgaacaagaattattggaattagataaatgggcaagtttgtggaattggtttaacataacaaattggctgtggtatataaaattattcataatgatagtaggaggcttggtaggtttaagaatagtttttgctgtactttctatagtgaatagagttaggcagggatattcaccattatcgtttcagacccacctcccaaccccgaggggacccgacaggcccgaaggaatagaagaagaaggtggagagagagacagagacagatccattcgattagtgaacggatctcgacggtatcgatgtcgacgataagctttgcaaagatggataaagttttaaacagagaggaatctttgcagctaatggaccttctaggtcttgaaaggagtgggaattggctccggtgcccgtcagtgggcagagcgcacatcgcccacagtccccgagaagttggggggaggggtcggcaattgaaccggtgcctagagaaggtggcgcggggtaaactgggaaagtgatgtcgtgtactggctccgcctttttcccgagggtgggggagaaccgtatataagtgcagtagtcgccgtgaacgttctttttcgcaacgggtttgccgccagaacacaggtaagtgccgtgtgtggttcccgcgggcctggcctctttacgggttatggcccttgcgtgccttgaattacttccactggctgcagtacgtgattcttgatcccgagcttcgggttggaagtgggtgggagagttcgaggccttgcgcttaaggagccccttcgcctcgtgcttgagttgaggcctggcctgggcgctggggccgccgcgtgcgaatctggtggcaccttcgcgcctgtctcgctgctttcgataagtctctagccatttaaaatttttgatgacctgctgcgacgctttttttctggcaagatagtcttgtaaatgcgggccaagatctgcacactggtatttcggtttttggggccgcgggcggcgacggggcccgtgcgtcccagcgcacatgttcggcgaggcggggcctgcgagcgcggccaccgagaatcggacgggggtagtctcaagctggccggcctgctctggtgcctggcctcgcgccgccgtgtatcgccccgccctgggcggcaaggctggcccggtcggcaccagttgcgtgagcggaaagatggccgcttcccggccctgctgcagggagctcaaaatggaggacgcggcgctcgggagagcgggcgggtgagtcacccacacaaaggaaaagggcctttccgtcctcagccgtcgcttcatgtgactccacggagtaccgggcgccgtccaggcacctcgattagttctcgagcttttggagtacgtcgtctttaggttggggggaggggttttatgcgatggagtttccccacactgagtgggtggagactgaagttaggccagcttggcacttgatgtaattctccttggaatttgccctttttgagtttggatcttggttcattctcaagcctcagacagtggttcaaagtttttttcttccatttcaggtgtcgtgaggaatttcgacatttaaatttaattaatctcgacggtatcggttaacttttaaaagaaaaggggggattggggggtacagtgcaggggaaagaatagtagacataatagcaacagacatacaaactaaagaattacaaaaacaaattacaaaaattcaaaattttatcgatcacgagactagcctcgaggtttatggctcagcggatgacaacacagctgctgctccttctagtgtgggtggctgtagtaggggaggctcagacaggagtgcaggtggagactatctccccaggagacgggcgcaccttccccaagcgcggccagacctgcgtggtgcactacaccgggatgcttgaagatggaaagaaatttgattcctcccgggacagaaacaagccctttaagtttatgctaggcaagcaggaggtgatccgaggctgggaagaaggggttgcccagatgagtgtgggtcagagagccaaactgactatatctccagattatgcctatggtgccactgggcacccaggcatcatcccaccacatgccactctcgtcttcgatgtggagcttctaaaactggaatctggcggtggatccaggattgcatgggccaggactgagcttctcaatgtctgcatgaacgccaagcaccacaaggaaaagccaggccccgaggacaagttgcatgagcagtgtcgaccctggaggaagaatgcctgctgttctaccaacaccagccaggaagcccataaggatgtttcctacctatatagattcaactggaaccactgtggagagatggcacctgcctgcaaacggcatttcatccaggacacctgcctctacgagtgctcccccaacttggggccctggatccagcaggtggatcagagctggcgcaaagagcgggtactgaacgtgcccctgtgcaaagaggactgtgagcaatggtgggaagattgtcgcacctcctacacctgcaagagcaactggcacaagggctggaactggacttcagggtttaacaagtgcgcagtgggagctgcctgccaacctttccatttctacttccccacacccactgttctgtgcaatgaaatctggactcactcctacaaggtcagcaactacagccgagggagtggccgctgcatccagatgtggttcgacccagcccagggcaaccccaatgaggaggtggcgaggttctatgctgcagccatgagtggggctgggccctgggcagcctggcctttcctgcttagcctggccctaatgctgctgtggctgctcagctgaaaactacgggctgcaggaattccgcccccccccccctaacgttactggccgaagccgcttggaataaggccggtgtgcgtttgtctatatgttattttccaccatattgccgtcttttggcaatgtgagggcccggaaacctggccctgtcttcttgacgagcattcctaggggtctttcccctctcgccaaaggaatgcaaggtctgttgaatgtcgtgaaggaagcagttcctctggaagcttcttgaagacaaacaacgtctgtagcgaccctttgcaggcagcggaaccccccacctggcgacaggtgcctctgcggccaaaagccacgtgtataagatacacctgcaaaggcggcacaaccccagtgccacgttgtgagttggatagttgtggaaagagtcaaatggctctcctcaagcgtattcaacaaggggctgaaggatgcccagaaggtaccccattgtatgggatctgatctggggcctcggtgcacatgctttacatgtgtttagtcgaggttaaaaaacgtctaggccccccgaaccacggggacgtggttttcctttgaaaaacacgatgataataccatggtgagcaagggcgaggagctgttcaccggggtggtgcccatcctggtcgagctggacggcgacgtaaacggccacaagttcagcgtgtccggcgagggcgagggcgatgccacctacggcaagctgaccctgaagttcatctgcaccaccggcaagctgcccgtgccctggcccaccctcgtgaccaccctgacctacggcgtgcagtgcttcagccgctaccccgaccacatgaagcagcacgacttcttcaagtccgccatgcccgaaggctacgtccaggagcgcaccatcttcttcaaggacgacggcaactacaagacccgcgccgaggtgaagttcgagggcgacaccctggtgaaccgcatcgagctgaagggcatcgacttcaaggaggacggcaacatcctggggcacaagctggagtacaactacaacagccacaacgtctatatcatggccgacaagcagaagaacggcatcaaggtgaacttcaagatccgccacaacatcgaggacggcagcgtgcagctcgccgaccactaccagcagaacacccccatcggcgacggccccgtgctgctgcccgacaaccactacctgagcacccagtccgccctgagcaaagaccccaacgagaagcgcgatcacatggtcctgctggagttcgtgaccgccgccgggatcactctcggcatggacgagctgtacaagtccggactcagatctcgactagctagtagctagctagctagtcgagctcaagcttcgaattcgatatcaagcttatcgcgataccgtcgacctcgagggaattccgataatcaacctctggattacaaaatttgtgaaagattgactggtattcttaactatgttgctccttttacgctatgtggatacgctgctttaatgcctttgtatcatgctattgcttcccgtatggctttcattttctcctccttgtataaatcctggttgctgtctctttatgaggagttgtggcccgttgtcaggcaacgtggcgtggtgtgcactgtgtttgctgacgcaacccccactggttggggcattgccaccacctgtcagctcctttccgggactttcgctttccccctccctattgccacggcggaactcatcgccgcctgccttgcccgctgctggacaggggctcggctgttgggcactgacaattccgtggtgttgtcggggaagctgacgtcctttccatggctgctcgcctgtgttgccacctggattctgcgcgggacgtccttctgctacgtcccttcggccctcaatccagcggaccttccttcccgcggcctgctgccggctctgcggcctcttccgcgtcttcgccttcgccctcagacgagtcggatctccctttgggccgcctccccgcatcgggaattcgagctcggtacctttaagaccaatgacttacaaggcagctgtagatcttagccactttttaaaagaaaaggggggactggaagggctaattcactcccaacgaagacaagatgggatcaattcaccatgggaataacttcgtatagcatacattatacgaagttatgctgctttttgcttgtactgggtctctctggttagaccagatctgagcctgggagctctctggctaactagggaacccactgcttaagcctcaataaagcttgccttgagtgcttcaagtagtgtgtgcccgtctgttgtgtgactctggtaactagagatccctcagacccttttagtcagtgtggaaaatctctagcagcatctagaattaattccgtgtattctatagtgtcacctaaatcgtatgtgtatgatacataaggttatgtattaattgtagccgcgttctaacgacaatatgtacaagcctaattgtgtagcatctggcttactgaagcagaccctatcatctctctcgtaaactgccgtcagagtcggtttggttggacgaaccttctgagtttctggtaacgccgtcccgcacccggaaatggtcagcgaaccaatcagcagggtcatcgctagccagatcctctacgccggacgcatcgtggccggcatcaccggcgccacaggtgcggttgctggcgcctatatcgccgacatcaccgatggggaagatcgggctcgccacttcgggctcatgagcgcttgtttcggcgtgggtatggtggcaggccccgtggccgggggactgttgggcgccatctccttgcatgcaccattccttgcggcggcggtgctcaacggcctcaacctactactgggctgcttcctaatgcaggagtcgcataagggagagcgtcgaatggtgcactctcagtacaatctgctctgatgccgcatagttaagccagccccgacacccgccaacacccgctgacgcgccctgacgggcttgtctgctcccggcatccgcttacagacaagctgtgaccgtctccgggagctgcatgtgtcagaggttttcaccgtcatcaccgaaacgcgcgagacgaaagggcctcgtgatacgcctatttttataggttaatgtcatgataataatggtttcttagacgtcaggtggcacttttcggggaaatgtgcgcggaacccctatttgtttatttttctaaatacattcaaatatgtatccgctcatgagacaataaccctgataaatgcttcaataatattgaaaaaggaagagtatgagtattcaacatttccgtgtcgcccttattcccttttttgcggcattttgccttcctgtttttgctcacccagaaacgctggtgaaagtaaaagatgctgaagatcagttgggtgcacgagtgggttacatcgaactggatctcaacagcggtaagatccttgagagttttcgccccgaagaacgttttccaatgatgagcacttttaaagttctgctatgtggcgcggtattatcccgtattgacgccgggcaagagcaactcggtcgccgcatacactattctcagaatgacttggttgagtactcaccagtcacagaaaagcatcttacggatggcatgacagtaagagaattatgcagtgctgccataaccatgagtgataacactgcggccaacttacttctgacaacgatcggaggaccgaaggagctaaccgcttttttgcacaacatgggggatcatgtaactcgccttgatcgttgggaaccggagctgaatgaagccataccaaacgacgagcgtgacaccacgatgcctgtagcaatggcaacaacgttgcgcaaactattaactggcgaactacttactctagcttcccggcaacaattaatagactggatggaggcggataaagttgcaggaccacttctgcgctcggcccttccggctggctggtttattgctgataaatctggagccggtgagcgtgggtctcgcggtatcattgcagcactggggccagatggtaagccctcccgtatcgtagttatctacacgacggggagtcaggcaactatggatgaacgaaatagacagatcgctgagataggtgcctcactgattaagcattggtaactgtcagaccaagtttactcatatatactttagattgatttaaaacttcatttttaatttaaaaggatctaggtgaagatcctttttgataatctcatgaccaaaatcccttaacgtgagttttcgttccactgagcgtcagaccccgtagaaaagatcaaaggatcttcttgagatcctttttttctgcgcgtaatctgctgcttgcaaacaaaaaaaccaccgctaccagcggtggtttgtttgccggatcaagagctaccaactctttttccgaaggtaactggcttcagcagagcgcagataccaaatactgtccttctagtgtagccgtagttaggccaccacttcaagaactctgtagcaccgcctacatacctcgctctgctaatcctgttaccagtggctgctgccagtggcgataagtcgtgtcttaccgggttggactcaagacgatagttaccggataaggcgcagcggtcgggctgaacggggggttcgtgcacacagcccagcttggagcgaacgacctacaccgaactgagatacctacagcgtgagcattgagaaagcgccacgcttcccgaagggagaaaggcggacaggtatccggtaagcggcagggtcggaacaggagagcgcacgagggagcttccagggggaaacgcctggtatctttatagtcctgtcgggtttcgccacctctgacttgagcgtcgatttttgtgatgctcgtcaggggggcggagcctatggaaaaacgccagcaacgcggcctttttacggttcctggccttttgctggccttttgctcacatgttctttcctgcgttatcccctgattctgtggataaccgtattaccgcctttgagtgagctgataccgctcgccgcagccgaacgaccgagcgcagcgagtcagtgagcgaggaagcggaagagcgcccaatacgcaaaccgcctctccccgcgcgttggccgattcattaatgcagctgtggaatgtgtgtcagttagggtgtggaaagtccccaggctccccagcaggcagaagtatgcaaagcatgcatctcaattagtcagcaaccaggtgtggaaagtccccaggctccccagcaggcagaagtatgcaaagcatgcatctcaattagtcagcaaccatagtcccgcccctaactccgcccatcccgcccctaactccgcccagttccgcccattctccgccccatggctgactaattttttttatttatgcagaggccgaggccgcctcggcctctgagctattccagaagtagtgaggaggcttttttggaggcctaggcttttgcaaaaagcttggacacaagacaggcttgcgagatatgtttgagaataccactttatcccgcgtcagggagaggcagtgcgtaaaaagacgcggactcatgtgaaatactggtttttagtgcgccagatctctataatctcgcgcaacctattttcccctcgaacactttttaagccgtagataaacaggctgggacacttcacatgagcgaaaaatacatcgtcacctgggacatgttgcagatccatgcacgtaaactcgcaagccgactgatgccttctgaacaatggaaaggcattattgccgtaagccgtggcggtctgtaccgggtgcgttactggcgcgtgaactgggtattcgtcatgtcgataccgtttgtatttccagctacgatcacgacaaccagcgcgagcttaaagtgctgaaacgcgcagaaggcgatggcgaaggcttcatcgttattgatgacctggtggataccggtggtactgcggttgcgattcgtgaaatgtatccaaaagcgcactttgtcaccatcttcgcaaaaccggctggtcgtccgctggttgatgactatgttgttgatatcccgcaagatacctggattgaacagccgtgggatatgggcgtcgtattcgtcccgccaatctccggtcgctaatcttttcaacgcctggcactgccgggcgttgttctttttaacttcaggcgggttacaatagtttccagtaagtattctggaggctgcatccatgacacaggcaaacctgagcgaaaccctgttcaaaccccgctttaaacatcctgaaacctcgacgctagtccgccgctttaatcacggcgcacaaccgcctgtgcagtcggcccttgatggtaaaaccatccctcactggtatcgcatgattaaccgtctgatgtggatctggcgcggcattgacccacgcgaaatcctcgacgtccaggcacgtattgtgatgagcgatgccgaacgtaccgacgatgatttatacgatacggtgattggctaccgtggcggcaactggatttatgagtgggccccggatctttgtgaaggaaccttacttctgtggtgtgacataattggacaaactacctacagagatttaaagctctaaggtaaatataaaatttttaagtgtataatgtgttaaactactgattctaattgtttgtgtattttagattccaacctatggaactgatgaatgggagcagtggtggaatgcctttaatgaggaaaacctgttttgctcagaagaaatgccatctagtgatgatgaggctactgctgactctcaacattctactcctccaaaaaagaagagaaaggtagaagaccccaaggactttccttcagaattgctaagttttttgagtcatgctgtgtttagtaatagaactcttgcttgctttgctatttacaccacaaaggaaaaagctgcactgctatacaagaaaattatggaaaaatattctgtaacctttataagtaggcataacagttataatcataacatactgttttttcttactccacacaggcatagagtgtctgctattaataactatgctcaaaaattgtgtacctttagctttttaatttgtaaaggggttaataaggaatatttgatgtatagtgccttgactagagatcataatcagccataccacatttgtagaggttttacttgctttaaaaaacctcccacacctccccctgaacctgaaacataaaatgaatgcaattgttgttgttaacttgtttattgcagcttataatggttacaaataaagcaatagcatcacaaatttcacaaataaagcatttttttcactgcattctagttgtggtttgtccaaactcatcaatgtatcttatcatgtctggatcaactggataactcaagctaaccaaaatcatcccaaacttcccaccccataccctattaccactgccaattacctagtggtttcatttactctaaacctgtgattcctctgaattattttcattttaaagaaattgtatttgttaaatatgtactacaaacttagtag

SEQ ID NO: 8 - DNA, 12182 bp, synthetic construct; identical to SEQ ID NO: 5
  misc_feature 1..12182: note = A synthetic pWPI mFKBP-mFRa SGGGS
  source 1..12182: mol_type = other DNA

SEQ ID NO: 9 - DNA, 10447 bp, synthetic construct
  misc_feature 1..10447: note = A synthetic pHR EcorI hAnti cd19 1D3 myc hinge cd28 cd3zeta
  source 1..10447: mol_type = other DNA
cgataccgtcgaccaaggcagctgtagatcttagccactttttaaaagaaaaggggggactggaagggctaattcactcccaacgaagacaagatctgctttttgcttgtactgggtctctctggttagaccagatctgagcctgggagctctctggctaactagggaacccactgcttaagcctcaataaagcttgccttgagtgcttcaagtagtgtgtgcccgtctgttgtgtgactctggtaactagagatccctcagacccttttagtcagtgtggaaaatctctagcagcatctagaattaattccgtgtattctatagtgtcacctaaatcgtatgtgtatgatacataaggttatgtattaattgtagccgcgttctaacgacaatatgtacaagcctaattgtgtagcatctggcttactgaagcagaccctatcatctctctcgtaaactgccgtcagagtcggtttggttggacgaaccttctgagtttctggtaacgccgtcccgcacccggaaatggtcagcgaaccaatcagcagggtcatcgctagccagatcctctacgccggacgcatcgtggccggcatcaccggcgccacaggtgcggttgctggcgcctatatcgccgacatcaccgatggggaagatcgggctcgccacttcgggctcatgagcgcttgtttcggcgtgggtatggtggcaggccccgtggccgggggactgttgggcgccatctccttgcatgcaccattccttgcggcggcggtgctcaacggcctcaacctactactgggctgcttcctaatgcaggagtcgcataagggagagcgtcgaatggtgcactctcagtacaatctagctctgatgccgcatagttaagccagccccgacacccgccaacacccgctgacgcgccctgacgggcttgtctgctcccggcatccgcttacagacaagctgtgaccgtctccgggagctgcatgtgtcagaggttttcaccgtcatcaccgaaacgcgcgagacgaaagggcctcgtgatacgcctatttttataggttaatgtcatgataataatggtttcttagacgtcaggtggcacttttcggggaaatgtgcgcggaacccctatttgtttatttttctaaatacattcaaatatgtatccgctcatgagacaataaccctgataaatgcttcaataatattgaaaaaggaagagtatgagtattcaacatttccgtgtcgcccttattcccttttttgcggcattttgccttcctgtttttgctcacccagaaacgctggtgaaagtaaaagatgctgaagatcagttgggtgcacgagtgggttacatcgaactggatctcaacagcggtaagatccttgagagttttcgccccgaagaacgttttccaatgatgagcacttttaaagttctgctatgtggcgcggtattatcccgtattgacgccgggcaagagcaactcggtcgccgcatacactattctcagaatgacttggttgagtactcaccagtcacagaaaagcatcttacggatggcatgacagtaagagaattatgcagtgctgccataaccatgagtgataacactgcggccaacttacttctgacaacgatcggaggaccgaaggagctaaccgcttttttgcacaacatgggggatcatgtaactcgccttgatcgttgggaaccggagctgaatgaagccataccaaacgacgagcgtgacaccacgatgcctgtagcaatggcaacaacgttgcgcaaactattaactggcgaactacttactctagcttcccggcaacaattaatagactggatggaggcggataaagttgcaggaccacttctgcgctcggcccttccggctggctggtttattgctgataaatctggagccggtgagcgtgggtctcgcggtatcattgcagcactggggccagatggtaagccctcccgtatcgtagttatctacacgacggggagtcaggcaactatggatgaacgaaatagacagatcgctgagataggtgcctcactgattaagcattggtaactgtcagaccaagtttactcatatatactttagattgatttaaaacttcatttttaatttaaaaggatctaggtgaagatcctttttgataatctcatgaccaaaatcccttaacgtgagttttcgttccactgagcgtcagaccccgtagaaaagatcaaaggatcttcttgagatcctttttttctgcgcgtaatctgctgcttgcaaacaaaaaaaccaccgctaccagcggtggtttgtttgccggatcaagagctaccaactctttttccgaaggtaactggcttcagcagagcgcagataccaaatactgtccttctagtgtagccgtagttaggccaccacttcaagaactctgtagcaccgcctacatacctcgctctgctaatcctgttaccagtggctgctgccagtggcgataagtcgtgtcttaccgggttggactcaagacgatagttaccggataaggcgcagcggtcgggctgaacggggggttcgtgcacacagcccagcttggagcgaacgacctacaccgaactgagatacctacagcgtgagctatgagaaagcgccacgcttcccgaagggagaaaggcggacaggtatccggtaagcggcagggtcggaacaggagagcgcacgagggagcttccagggggaaacgcctggtatctttatagtcctgtcgggtttcgccacctctgacttgagcgtcgatttttgtgatgctcgtcaggggggcggagcctatggaaaaacgccagcaacgcggcctttttacggttcctggccttttgctggccttttgctcacatgttctttcctgcgttatcccctgattctgtggataaccgtattaccgcctttgagtgagctgataccgctcgccgcagccgaacgaccgagcgcagcgagtcagtgagcgaggaagcggaagagcgcccaatacgcaaaccgcctctccccgcgcgttggccgattcattaatgcagctgtggaatgtgtgtcagttagggtgtggaaagtccccaggctccccagcaggcagaagtatgcaaagcatgcatctcaattagtcagcaaccaggtgtggaaagtccccaggctccccagcaggcagaagtatgcaaagcatgcatctcaattagtcagcaaccatagtcccgcccctaactccgcccatcccgcccctaactccgcccagttccgcccattctccgccccatggctgactaattttttttatttatgcagaggccgaggccgcctcggcctctgagctattccagaagtagtgaggaggcttttttggaggcctaggcttttgcaaaaagcttggacacaagacaggcttgcgagatatgtttgagaataccactttatcccgcgtcagggagaggcagtgcgtaaaaagacgcggactcatgtgaaatactggtttttagtgcgccagatctctataatctcgcgcaacctattttcccctcgaacactttttaagccgtagataaacaggctgggacacttcacatgagcgaaaaatacatcgtcacctgggacatgttgcagatccatgcacgtaaactcgcaagccgactgatgccttctgaacaatggaaaggcattattgccgtaagccgtggcggtctgtaccgggtgcgttactggcgcgtgaactgggtattcgtcatgtcgataccgtttgtatttccagctacgatcacgacaaccagcgcgagcttaaagtgctgaaacgcgcagaaggcgatggcgaaggcttcatcgttattgatgacctggtggataccggtggtactgcggttgcgattcgtgaaatgtatccaaaagcgcactttgtcaccatcttcgcaaaaccggctggtcgtccgctggttgatgactatgttgttgatatcccgcaagatacctggattgaacagccgtgggatatgggcgtcgtattcgtcccgccaatctccggtcgctaatcttttcaacgcctggcactgccgggcgttgttctttttaacttcaggcgggttacaatagtttccagtaagtattctggaggctgcatccatgacacaggcaaacctgagcgaaaccctgttcaaaccccgctttaaacatcctgaaacctcgacgctagtccgccgctttaatcacggcgcacaaccgcctgtgcagtcggcccttgatggtaaaaccatccctcactggtatcgcatgattaaccgtctgatgtggatctggcgcggcattgacccacgcgaaatcctcgacgtccaggcacgtattgtgatgagcgatgccgaacgtaccgacgatgatttatacgatacggtgattggctaccgtggcggcaactggatttatgagtgggccccggatctttgtgaaggaaccttacttctgtggtgtgacataattggacaaactacctacagagatttaaagctctaaggtaaatataaaatttttaagtgtataatgtgttaaactactgattctaattgtttgtgtattttagattccaacctatggaactgatgaatgggagcagtggtggaatgcctttaatgaggaaaacctgttttgctcagaagaaatgccatctagtgatgatgaggctactgctgactctcaacattctactcctccaaaaaagaagagaaaggtagaagaccccaaggactttccttcagaattgctaagttttttgagtcatgctgtgtttagtaatagaactcttgcttgctttgctatttacaccacaaaggaaaaagctgcactgctatacaagaaaattatggaaaaatattctgtaacctttataagtaggcataacagttataatcataacatactgttttttcttactccacacaggcatagagtgtctgctattaataactatgctcaaaaattgtgtacctttagctttttaatttgtaaaggggttaataaggaatatttgatgtatagtgccttgactagagatcataatcagccataccacatttgtagaggttttacttgctttaaaaaacctcccacacctccccctgaacctgaaacataaaatgaatgcaattgttgttgttaacttgtttattgcagcttataatggttacaaataaagcaatagcatcacaaatttcacaaataaagcatttttttcactgcattctagttgtggtttgtccaaactcatcaatgtatcttatcatgtctggatcaactggataactcaagctaaccaaaatcatcccaaacttcccaccccataccctattaccactgccaattacctagtggtttcatttactctaaacctgtgattcctctgaattattttcattttaaagaaattgtatttgttaaatatgtactacaaacttagtagttggaagggctaattcactcccaaagaagacaagatatccttgatctgtggatctaccacacacaaggctacttccctgattagcagaactacacaccagggccaggggtcagatatccactgacctttggatggtgctacaagctagtaccagttgagccagataaggtagaagaggccaataaaggagagaacaccagcttgttacaccctgtgagcctgcatgggatggatgacccggagagagaagtgttagagtggaggtttgacagccgcctagcatttcatcacgtggcccgagagctgcatccggagtacttcaagaactgctgatatcgagcttgctacaagggactttccgctggggactttccagggaggcgtggcctgggcgggactggggagtggcgagccctcagatcctgcatataagcagctgctttttgcctgtactgggtctctctggttagaccagatctgagcctgggagctctctggctaactagggaacccactgcttaagcctcaataaagcttgccttgagtgcttcaagtagtgtgtgcccgtctgttgtgtgactctggtaactagagatccctcagacccttttagtcagtgtggaaaatctctagcagtggcgcccgaacagggacttgaaagcgaaagggaaaccagaggagctctctcgacgcaggactcggcttgctgaagcgcgcacggcaagaggcgaggggcggcgactggtgagtacgccaaaaattttgactagcggaggctagaaggagagagatgggtgcgagagcgtcagtattaagcgggggagaattagatcgcgatgggaaaaaattcggttaaggccagggggaaagaaaaaatataaattaaaacatatagtatgggcaagcagggagctagaacgattcgcagttaatcctggcctgttagaaacatcagaaggctgtagacaaatactgggacagctacaaccatcccttcagacaggatcagaagaacttagatcattatataatacagtagcaaccctctattgtgtgcatcaaaggatagagataaaagacaccaaggaagctttagacaagatagaggaagagcaaaacaaaagtaagaccaccgcacagcaagcggccggtgatcttcagacctggacgatatatatgagggacaattggagaagtgaattatataaatataaagtagtaaaaattgaaccattaggagtagcacccaccaaggcaaagagaagagtggtgcagagagaaaaaagagcagtgggaataggagctttgttccttgggttcttgggagcagcaggaagcactatgggcgcagcgtcaatgacgctgacggtacaggccagacaattattgtctggtatagtgcagcagcagaacaatttgctgagggctattgaggcgcaacagcatctgttgcaactcacagtctggggcatcaagcagctccaggcaagaatcctggctgtggaaagatacctaaaggatcaacagctcctggggatttggggttgctctggaaaactcatttgcaccactgctgtgccttggaatgctagttggagtaataaatctctggaacagatttggaatcacacgacctggatggagtgggacagagaaattaacaattacacaagcttaatacactccttaattgaagaatcgcaaaaccagcaagaaaagaatgaacaagaattattggaattagataaatgggcaagtttgtggaattggtttaacataacaaattggctgtggtatataaaattattcataatgatagtaggaggcttggtaggtttaagaatagtttttgctgtactttctatagtgaatagagttaggcagggatattcaccattatcgtttcagacccacctcccaaccccgaggggacccgacaggcccgaaggaatagaagaagaaggtggagagagagacagagacagatccattcgattagtgaacggatctcgacggtcgccaaatggcagtattcatccacaattttaaaagaaaaggggggattggggggtacagtgcaggggaaagaatagtagacataatagcaacagacatacaaactaaagaattacaaaaacaaattacaaaaattcaaaattttcgggtttattacagggacagcagagatccagtttggatcgataagcttgatatcgaattgggtaggggaggcgcttttcccaaggcagtctggagcatgcgctttagcagccccgctgggcacttggcgctacacaagtggcctctggcctcgcacacattccacatccaccggtaggcgccaaccggctccgttctttggtggccccttcgcgccaccttctactcctcccctagtcaggaagttcccccccgccccgcagctcgcgtcgtgcaggacgtgacaaatggaagtagcacgtctcactagtctcgtgcagatggacagcaccgctgagcaatggaagcgggtaggcctttggggcagcggccaatagcagctttgctccttcgctttctgggctcagaggctgggaaggggtgggtccgggggcgggctcaggggcgggctcaggggcggggcgggcgcccgaaggtcctccggaggcccggcattctgcacgcttcaaaagcgcacgtctgccgcgctgttctcctcttcctcatctccgggcctttcgatggctcttccagtgactgctcttctcctcccgcttgcgctgctgttgcatgcggctcggccggagcaaaagctgatttcagaagaggacttggatatccagatgacacagaccacttcatctctttctgctagcctgggggatcgggtcacaataagctgtcgcgcatcccaagacataagcaaatatctgaattggtatcaacagaaacccgatggaactgtgaaacttctcatctaccatacgagcagactgcattctggggttcctagccgcttttcagggtctggatctggaacggactattcacttaccatatctaatttggaacaagaagacatcgcgacctatttctgtcagcaaggcaatacgctcccttatacttttggagggggaacgaagttggagatcacaggtggaggcggcagtggcgggggaggatctggtggaggtggttctgaggtcaagctgcaggagagtggtcccgggctggtagccccgagccagagtctgtctgttacttgcactgtgtcaggcgtgagtctcccagactatggtgtatcatggattcgacagccgccccggaaaggacttgagtggctcggagtgatctggggatccgaaacgacgtactacaatagcgcgctcaaaagccggctgaccatcattaaggataactctaaaagccaggtgttcttgaaaatgaattccttgcagacagatgatacggcgatctattactgtgccaagcactactactatggaggcagctatgccatggattattggggtcaaggcacttctgtgacagtgagcagtgccgcagctattgaagtgatgtacccgcctccgtatcttgataatgagaaatctaacggaaccataatacacgtgaaaggcaaacatttgtgtccgtctcctctgttccccgggcctagtaaaccgttttgggtactggtggtggtaggcggagtacttgcatgttactcactcctcgttaccgtcgcattcattatcttctgggtacggagcaagagatctcggctgcttcatagcgattatatgaatatgacacccagacgcccaggtcctactaggaaacattaccagccgtatgcgccgccgagggacttcgccgcatacagatctcgcgtgaagttctcaagatctgccgatgcaccggcttatcagcagggacaaaaccaactgtataatgagctgaacctggggcggagggaggagtatgatgtcctggacaagcgaagagggcgagaccccgaaatgggaggcaagcctcaacggcggaagaacccacaagagggcctgtataacgagcttcaaaaggacaaaatggcggaagcgtatagcgagatcggaatgaagggcgaacgaaggagagggaaaggtcacgatgggctctaccaggggctcagcacggcaacaaaagacacatatgacgcattgcatatgcaggcgctgccaccgagatgactcacgcgtcaagtggagcaaggcaggtggacagtggatccttgacttgcggccgcaactcccacctgcaacatgcgtgactgactgaggccgcgactctagagtcgacctgcaggcatgcaagcttgatatcaagcttatcgataatcaacctctggattacaaaatttgtgaaagattgactggtattcttaactatgttgctccttttacgctatgtggatacgctgctttaatgcctttgtatcatgctattgcttcccgtatggctttcattttctcctccttgtataaatcctggttgctgtctctttatgaggagttgtggcccgttgtcaggcaacgtggcgtggtgtgcactgtgtttgctgacgcaacccccactggttggggcattgccaccacctgtcagctcctttccgggactttcgctttccccctccctattgccacggcggaactcatcgccgcctgccttgcccgctgctggacaggggctcggctgttgggcactgacaattccgtggtgttgtcggggaaatcatcgtcctttccttggctgctcgcctgtgttgccacctggattctgcgcgggacgtccttctgctacgtcccttcggccctcaatccagcggaccttccttcccgcggcctgctgccggctctgcggcctcttccgcgtcttcgccttcgccctcagacgagtcggatctccctttgggccgcctccccgcat

SEQ ID NO: 10 - DNA, 12536 bp, synthetic construct
  misc_feature 1..12536: note = A synthetic pWPI pmei mAnti cd19 1D3 myc hinge cd28 cd3zeta
  source 1..12536: mol_type = other DNA
ttggaagggctaattcactcccaaagaagacaagatatccttgatctgtggatctaccacacacaaggctacttccctgattagcagaactacacaccagggccaggggtcagatatccactgacctttggatggtgctacaagctagtaccagttgagccagataaggtagaagaggccaataaaggagagaacaccagcttgttacaccctgtgagcctgcatgggatggatgacccggagagagaagtgttagagtggaggtttgacagccgcctagcatttcatcacgtggcccgagagctgcatccggagtacttcaagaactgctgatatcgagcttgctacaagggactttccgctggggactttccagggaggcgtggcctgggcgggactggggagtggcgagccctcagatcctgcatataagcagctgctttttgcctgtactgggtctctctggttagaccagatctgagcctgggagctctctggctaactagggaacccactgcttaagcctcaataaagcttgccttgagtgcttcaagtagtgtgtgcccgtctgttgtgtgactctggtaactagagatccctcagacccttttagtcagtgtggaaaatctctagcagtggcgcccgaacagggacttgaaagcgaaagggaaaccagaggagctctctcgacgcaggactcggcttgctgaagcgcgcacggcaagaggcgaggggcggcgactggtgagtacgccaaaaattttgactagcggaggctagaaggagagagatgggtgcgagagcgtcagtattaagcgggggagaattagatcgcgatgggaaaaaattcggttaaggccagggggaaagaaaaaatataaattaaaacatatagtatgggcaagcagggagctagaacgattcgcagttaatcctggcctgttagaaacatcagaaggctgtagacaaatactgggacagctacaaccatcccttcagacaggatcagaagaacttagatcattatataatacagtagcaaccctctattgtgtgcatcaaaggatagagataaaagacaccaaggaagctttagacaagatagaggaagagcaaaacaaaagtaagaccaccgcacagcaagcggccgctgatcttcagacctggaggaggagatatgagggacaattggagaagtgaattatataaatataaagtagtaaaaattgaaccattaggagtagcacccaccaaggcaaagagaagagtggtgcagagagaaaaaagagcagtgggaataggagctttgttccttgggttcttgggagcagcaggaagcactatgggcgcagcgtcaatgacgctgacggtacaggccagacaattattgtctggtatagtgcagcagcagaacaatttgctgagggctattgaggcgcaacagcatctgttgcaactcacagtctggggcatcaagcagctccaggcaagaatcctggctgtggaaagatacctaaaggatcaacagctcctggggatttggggttgctctggaaaactcatttgcaccactgctgtgccttggaatgctagttggagtaataaatctctggaacagatttggaatcacacgacctggatggagtgggacagagaaattaacaattacacaagcttaatacactccttaattgaagaatcgcaaaaccagcaagaaaagaatgaacaagaattattggaattagataaatgggcaagtttgtggaattggtttaacataacaaattggctgtggtatataaaattattcataatgatagtaggaggcttggtaggtttaagaatagtttttgctgtactttctatagtgaatagagttaggcagggatattcaccattatcgtttcagacccacctcccaaccccgaggggacccgacaggcccgaaggaatagaagaagaaggtggagagagagacagagacagatccattcgattagtgaacggatctcgacggtatcgatgtcgacgataagctttgcaaagatggataaagttttaaacagagaggaatctttgcagctaatggaccttctaggtcttgaaaggagtgggaattggctccggtgcccgtcagtgggcagagcgcacatcgcccacagtccccgagaagttggggggaggggtcggcaattgaaccggtgcctagagaaggtggcgcggggtaaactgggaaagtgatgtcgtgtactggctccgcctttttcccgagggtgggggagaaccgtatataagtgcagtagtcgccgtgaacgttctttttcgcaacgggtttgccgccagaacacaggtaagtgccgtgtgtggttcccgcgggcctggcctctttacgggttatggcccttgcgtgccttgaattacttccactggctgcagtacgtgattcttgatcccgagcttcgggttggaagtgggtgggagagttcgaggccttgcgcttaaggagccccttcgcctcgtgcttgagttgaggcctggcctgggcgctggggccgccgcgtgcgaatctggtggcaccttcgcgcctgtctcgctgctttcgataagtctctagccatttaaaatttttgatgacctgctgcgacgctttttttctggcaagatagtcttgtaaatgcgggccaagatctgcacactggtatttcggtttttggggccgcgggcggcgacggggcccgtgcgtcccagcgcacatgttcggcgaggcggggcctgcgagcgcggccaccgagaatcggacgggggtagtctcaagctggccggcctgctctggtgcctggcctcgcgccgccgtgtatcgccccgccctgggcggcaaggctggcccggtcggcaccagttgcgtgagcggaaagatggccgcttcccggccctgctgcagggagctcaaaatggaggacgcggcgctcgggagagcgggcgggtgagtcacccacacaaaggaaaagggcctttccgtcctcagccgtcgcttcatgtgactccacggagtaccgggcgccgtccaggcacctcgattagttctcgagcttttggagtacgtcgtctttaggttggggggaggggttttatgcgatggagtttccccacactgagtgggtggagactgaagttaggccagcttggcacttgatgtaattctccttggaatttgccctttttgagtttggatcttggttcattctcaagcctcagacagtggttcaaagtttttttcttccatttcaggtgtcgtgaggaatttcgacatttaaatttaattaatctcgacggtatcggttaacttttaaaagaaaaggggggattggggggtacagtgcaggggaaagaatagtagacataatagcaacagacatacaaactaaagaattacaaaaacaaattacaaaaattcaaaattttatcgatcacgagactagcctcgaggtttatgggggttcccacccagctgttggggttgctgctcctctggatcactgatgccatctgcgaacagaagctcatttctgaagaagatctggacatacagatgacccagagtcctgccagcttgtccacatccctcggagagaccgtgacaattcaatgccaggcctctgaggacatatattctggattggcttggtaccagcaaaagccaggtaaaagtcctcagttgttgatatacggcgcttctgatttgcaagacggggtgccctcacgatttagcgggtctggaagtggcactcagtacagtctgaagattacttcaatgcaaacagaagacgagggtgtgtatttttgccaacaggggctgacctacccaaggacattcgggggcggtacaaagcttgaacttaagggcggcggtgggtctggaggtggtggatctggcggagggggaagtgaggtacagctgcaacagtccggcgccgaactcgttcgccctggaacctcagtcaaattgtcatgcaaggtgagtggcgacacaataaccttttactatatgcacttcgttaaacagaggccaggtcaaggtctggaatggataggcagaattgatccagaagatgagtccaccaaatactcagaaaagttcaaaaacaaagccactcttactgccgacacctcaagcaacacagcatatcttaagctcagttcacttaccagcgaagacaccgccacctatttttgtatttatggtggctattactttgactactgggggcaaggtgttatggtaacagtttcttccattgaattcatgtatccacccccctatttggataatgaacgatctaatgggactataatacatatcaaggaaaagcatctgtgtcatacccaaagttcccctaagcttttctgggccctcgtcgttgtggcaggagtgcttttttgctatggattgttggttactgtggctctctgcgtcatttggacaaatagtaggaggaatcgggggggacaatctgattacatgaacatgacaccacggaggccaggccttaccagaaagccctaccaaccttatgcaccagcacgagacttcgccgcatacaggccaagggctaagttttcccgcagcgccgaaaccgcagccaacctccaagatcctaatcagctctataacgaattgaatcttggccgcagagaggagtacgacgtacttgagaaaaagagagctagggaccctgaaatgggtgggaagcaacagcgaagaaggaacccacaggaaggggtgtataatgcccttcaaaaggataaaatggcagaggcatacagtgaaatcggaaccaagggggagagacgcagagggaaaggccatgacggcctttatcagggtttgtcaactgctactaaagacacttatgatgccttgcatatgcaaactctcgcacccagatgaaaactacgggctgcaggaattccgcccccccccccctaacgttactggccgaagccgcttggaataaggccggtgtgcgtttgtctatatgttattttccaccatattgccgtcttttggcaatgtgagggcccggaaacctggccctgtcttcttgacgagcattcctaggggtctttcccctctcgccaaaggaatgcaaggtctgttgaatgtcgtgaaggaagcagttcctctggaagcttcttgaagacaaacaacgtctgtagcgaccctttgcaggcagcggaaccccccacctggcgacaggtgcctctgcggccaaaagccacgtgtataagatacacctgcaaaggcggcacaaccccagtgccacgttgtgagttggatagttgtggaaagagtcaaatggctctcctcaagcgtattcaacaaggggctgaaggatgcccagaaggtaccccattgtatgggatctgatctggggcctcggtgcacatgctttacatgtgtttagtcgaggttaaaaaacgtctaggccccccgaaccacggggacgtggttttcctttgaaaaacacgatgataataccatggtgagcaagggcgaggagctgttcaccggggtggtgcccatcctggtcgagctggacggcgacgtaaacggccacaagttcagcgtgtccggcgagggcgagggcgatgccacctacggcaagctgaccctgaagttcatctgcaccaccggcaagctgcccgtgccctggcccaccctcgtgaccaccctgacctacggcgtgcagtgcttcagccgctaccccgaccacatgaagcagcacgacttcttcaagtccgccatgcccgaaggctacgtccaggagcgcaccatcttcttcaaggacgacggcaactacaagacccgcgccgaggtgaagttcgagggcgacaccctggtgaaccgcatcgagctgaagggcatcgacttcaaggaggacggcaacatcctggggcacaagctggagtacaactacaacagccacaacgtctatatcatggccgacaagcagaagaacggcatcaaggtgaacttcaagatccgccacaacatcgaggacggcagcgtgcagctcgccgaccactaccagcagaacacccccatcggcgacggccccgtgctgctgcccgacaaccactacctgagcacccagtccgccctgagcaaagaccccaacgagaagcgcgatcacatggtcctgctggagttcgtgaccgccgccgggatcactctcggcatggacgagctgtacaagtccggactcagatctcgactagctagtagctagctagctagtcgagctcaagcttcgaattcgatatcaagcttatcgcgataccgtcgacctcgagggaattccgataatcaacctctggattacaaaatttgtgaaagattgactggtattcttaactatgttgctccttttacgctatgtggatacgctgctttaatgcctttgtatcatgctattgcttcccgtatggctttcattttctcctccttgtataaatcctggttgctgtctctttatgaggagttgtggcccgttgtcaggcaacgtggcgtggtgtgcactgtgtttgctgacgcaacccccactggttggggcattgccaccacctgtcagctcctttccgggactttcgctttccccctccctattgccacggcggaactcatcgccgcctgccttgcccgctgctggacaggggctcggctgttgggcactgacaattccgtggtgttgtcggggaagctgacgtcctttccatggctgctcgcctgtgttgccacctggattctgcgcgggacgtccttctgctacgtcccttcggccctcaatccagcggaccttccttcccgcggcctgctgccggctctgcggcctcttccgcgtcttcgccttcgccctcagacgagtcggatctccctttgggccgcctccccgcatcgggaattcgagctcggtacctttaagaccaatgacttacaaggcagctgtagatcttagccactttttaaaagaaaaggggggactggaagggctaattcactcccaacgaagacaagatgggatcaattcaccatgggaataacttcgtatagcatacattatacgaagttatgctgctttttgcttgtactgggtctctctggttagaccagatctgagcctgggagctctctggctaactagggaacccactgcttaagcctcaataaagcttgccttgagtgcttcaagtagtgtgtgcccgtctgttgtgtgactctggtaactagagatccctcagacccttttagtcagtgtggaaaatctctagcagcatctagaattaattccgtgtattctatagtgtcacctaaatcgtatgtgtatgatacataaggttatgtattaattgtagccgcgttctaacgacaatatgtacaagcctaattgtgtagcatctggcttactgaagcagaccctatcatctctctcgtaaactgccgtcagagtcggtttggttggacgaaccttctgagtttctggtaacgccgtcccgcacccggaaatggtcagcgaaccaatcagcagggtcatcgctagccagatcctctacgccggacgcatcgtggccggcatcaccggcgccacaggtgcggttgctggcgcctatatcgccgacatcaccgatggggaagatcgggctcgccacttcgggctcatgagcgcttgtttcggcgtgggtatggtggcaggccccgtggccgggggactgttgggcgccatctccttgcatgcaccattccttgcggcggcggtgctcaacggcctcaacctactactgggctgcttcctaatgcaggagtcgcataagggagagcgtcgaatggtgcactctcagtacaatctgctctgatgccgcatagttaagccagccccgacacccgccaacacccgctgacgcgccctgacgggcttgtctgctcccggcatccgcttacagacaagctgtgaccgtctccgggagctgcatgtgtcagaggttttcaccgtcatcaccgaaacgcgcgagacgaaagggcctcgtgatacgcctatttttataggttaatgtcatgataataatggtttcttagacgtcaggtggcacttttcggggaaatgtgcgcggaacccctatttgtttatttttctaaatacattcaaatatgtatccgctcatgagacaataaccctgataaatgcttcaataatattgaaaaaggaagagtatgagtattcaacatttccgtgtcgcccttattcccttttttgcggcattttgccttcctgtttttgctcacccagaaacgctggtgaaagtaaaagatgctgaagatcagttgggtgcacgagtgggttacatcgaactggatctcaacagcggtaagatccttgagagttttcgccccgaagaacgttttccaatgatgagcacttttaaagttctgctatgtggcgcggtattatcccgtattgacgccgggcaagagcaactcggtcgccgcatacactattctcagaatgacttggttgagtactcaccagtcacagaaaagcatcttacggatggcatgacagtaagagaattatgcagtgctgccataaccatgagtgataacactgcggccaacttacttctgacaacgatcggaggaccgaaggagctaaccgcttttttgcacaacatgggggatcatgtaactcgccttgatcgttgggaaccggagctgaatgaagccataccaaacgacgagcgtgacaccacgatgcctgtagcaatggcaacaacgttgcgcaaactattaactggcgaactacttactctagcttcccggcaacaattaatagactggatggaggcggataaagttgcaggaccacttctgcgctcggcccttccggctggctggtttattgctgataaatctggagccggtgagcgtgggtctcgcggtatcattgcagcactggggccagatggtaagccctcccgtatcgtagttatctacacgacggggagtcaggcaactatggatgaacgaaatagacagatcgctgagataggtgcctcactgattaagcattggtaactgtcagaccaagtttactcatatatactttagattgatttaaaacttcatttttaatttaaaaggatctaggtgaagatcctttttgataatctcatgaccaaaatcccttaacgtgagttttcgttccactgagcgtcagaccccgtagaaaagatcaaaggatcttcttgagatcctttttttctgcgcgtaatctgctgcttgcaaacaaaaaaaccaccgctaccagcggtggtttgtttgccggatcaagagctaccaactctttttccgaaggtaactggcttcagcagagcgcagataccaaatactgtccttctagtgtagccgtagttaggccaccacttcaagaactctgtagcaccgcctacatacctcgctctgctaatcctgttaccagtggctgctgccagtggcgataagtcgtgtcttaccgggttggactcaagacgatagttaccggataaggcgcagcggtcgggctgaacggggggttcgtgcacacagcccagcttggagcgaacgacctacaccgaactgagatacctacagcgtgagcattgagaaagcgccacgcttcccgaagggagaaaggcggacaggtatccggtaagcggcagggtcggaacaggagagcgcacgagggagcttccagggggaaacgcctggtatctttatagtcctgtcgggtttcgccacctctgacttgagcgtcgatttttgtgatgctcgtcaggggggcggagcctatggaaaaacgccagcaacgcggcctttttacggttcctggccttttgctggccttttgctcacatgttctttcctgcgttatcccctgattctgtggataaccgtattaccgcctttgagtgagctgataccgctcgccgcagccgaacgaccgagcgcagcgagtcagtgagcgaggaagcggaagagcgcccaatacgcaaaccgcctctccccgcgcgttggccgattcattaatgcagctgtggaatgtgtgtcagttagggtgtggaaagtccccaggctccccagcaggcagaagtatgcaaagcatgcatctcaattagtcagcaaccaggtgtggaaagtccccaggctccccagcaggcagaagtatgcaaagcatgcatctcaattagtcagcaaccatagtcccgcccctaactccgcccatcccgcccctaactccgcccagttccgcccattctccgccccatggctgactaattttttttatttatgcagaggccgaggccgcctcggcctctgagctattccagaagtagtgaggaggcttttttggaggcctaggcttttgcaaaaagcttggacacaagacaggcttgcgagatatgtttgagaataccactttatcccgcgtcagggagaggcagtgcgtaaaaagacgcggactcatgtgaaatactggtttttagtgcgccagatctctataatctcgcgcaacctattttcccctcgaacactttttaagccgtagataaacaggctgggacacttcacatgagcgaaaaatacatcgtcacctgggacatgttgcagatccatgcacgtaaactcgcaagccgactgatgccttctgaacaatggaaaggcattattgccgtaagccgtggcggtctgtaccgggtgcgttactggcgcgtgaactgggtattcgtcatgtcgataccgtttgtatttccagctacgatcacgacaaccagcgcgagcttaaagtgctgaaacgcgcagaaggcgatggcgaaggcttcatcgttattgatgacctggtggataccggtggtactgcggttgcgattcgtgaaatgtatccaaaagcgcactttgtcaccatcttcgcaaaaccggctggtcgtccgctggttgatgactatgttgttgatatcccgcaagatacctggattgaacagccgtgggatatgggcgtcgtattcgtcccgccaatctccggtcgctaatcttttcaacgcctggcactgccgggcgttgttctttttaacttcaggcgggttacaatagtttccagtaagtattctggaggctgcatccatgacacaggcaaacctgagcgaaaccctgttcaaaccccgctttaaacatcctgaaacctcgacgctagtccgccgctttaatcacggcgcacaaccgcctgtgcagtcggcccttgatggtaaaaccatccctcactggtatcgcatgattaaccgtctgatgtggatctggcgcggcattgacccacgcgaaatcctcgacgtccaggcacgtattgtgatgagcgatgccgaacgtaccgacgatgatttatacgatacggtgattggctaccgtggcggcaactggatttatgagtgggccccggatctttgtgaaggaaccttacttctgtggtgtgacataattggacaaactacctacagagatttaaagctctaaggtaaatataaaatttttaagtgtataatgtgttaaactactgattctaattgtttgtgtattttagattccaacctatggaactgatgaatgggagcagtggtggaatgcctttaatgaggaaaacctgttttgctcagaagaaatgccatctagtgatgatgaggctactgctgactctcaacattctactcctccaaaaaagaagagaaaggtagaagaccccaaggactttccttcagaattgctaagttttttgagtcatgctgtgtttagtaatagaactcttgcttgctttgctatttacaccacaaaggaaaaagctgcactgctatacaagaaaattatggaaaaatattctgtaacctttataagtaggcataacagttataatcataacatactgttttttcttactccacacaggcatagagtgtctgctattaataactatgctcaaaaattgtgtacctttagctttttaatttgtaaaggggttaataaggaatatttgatgtatagtgccttgactagagatcataatcagccataccacatttgtagaggttttacttgctttaaaaaacctcccacacctccccctgaacctgaaacataaaatgaatgcaattgttgttgttaacttgtttattgcagcttataatggttacaaataaagcaatagcatcacaaatttcacaaataaagcatttttttcactgcattctagttgtggtttgtccaaactcatcaatgtatcttatcatgtctggatcaactggataactcaagctaaccaaaatcatcccaaacttcccaccccataccctattaccactgccaattacctagtggtttcatttactctaaacctgtgattcctctgaattattttcattttaaagaaattgtatttgttaaatatgtactacaaacttagtag

SEQ ID NO: 11 - protein, 365 aa, synthetic construct
  REGION 1..365: note = A synthetic FKBP-1SG-FR with GPI anchor amino acid sequence
MTTQLLLLLVWVAVVGEAQTGVQVETISPGDGRTFPKRGQTCVVHYTGMLEDGKKFDSSRDRNKPFKFMLGKQEVIRGWEEGVAQMSVGQRAKLTISPDYAYGATGHPGIIPPHATLVFDVELLKLESGGGSRIAWARTELLNVCMNAKHHKEKPGPEDKLHEQCRPWRKNACCSTNTSQEAHKDVSYLYRFNWNHCGEMAPACKRHFIQDTCLYECSPNLGPWIQQVDQSWRKERVLNVPLCKEDCEQWWEDCRTSYTCKSNWHKGWNWTSGFNKCAVGAACQPFHFYFPTPTVLCNEIWTHSYKVSNYSRGSGRCIQMWFDPAQGNPNEEVARFYAAAMSGAGPWAAWPFLLSLALMLLWLLS

SEQ ID NO: 12 - protein, 375 aa, synthetic construct
  REGION 1..375: note = A synthetic FKBP-3SG-FR with GPI anchor amino acid sequence
MTTQLLLLLVWVAVVGEAQTGVQVETISPGDGRTFPKRGQTCVVHYTGMLEDGKKFDSSRDRNKPFKFMLGKQEVIRGWEEGVAQMSVGQRAKLTISPDYAYGATGHPGIIPPHATLVFDVELLKLEGGGGSGGGGSGGGGSRIAWARTELLNVCMNAKHHKEKPGPEDKLHEQCRPWRKNACCSTNTSQEAHKDVSYLYRFNWNHCGEMAPACKRHFIQDTCLYECSPNLGPWIQQVDQSWRKERVLNVPLCKEDCEQWWEDCRTSYTCKSNWHKGWNWTSGFNKCAVGAACQPFHFYFPTPTVLCNEIWTHSYKVSNYSRGSGRCIQMWFDPAQGNPNEEVARFYAAAMSGAGPWAAWPFLLSLALMLLWLLS

SEQ ID NO: 13 - protein, 513 aa, synthetic construct
  REGION 1..513: note = A synthetic 4M5.3-FR with GPI anchor amino acid sequence
MALPVTALLLPLALLLHAARPDVVMTQTPLSLPVSLGDQASISCRSSQSLVHSNGNTYLRWYLQKPGQSPKVLIYKVSNRVSGVPDRFSGSGSGTDFTLKINRVEAEDLGVYFCSQSTHVPWTFGGGTKLEIKSSADDAKKDAAKKDDAKKDDAKKDGGVKLDETGGGLVQPGGAMKLSCVTSGFTFGHYWMNWVRQSPEKGLEWVAQFRNKPYNYETYYSDSVKGRFTISRDDSKSSVYLQMNNLRVEDTGIYYCTGASYGMEYLGQGTSVTVSSGGGSRIAWARTELLNVCMNAKHHKEKPGPEDKLHEQCRPWRKNACCSTNTSQEAHKDVSYLYRFNWNHCGEMAPACKRHFIQDTCLYECSPNLGPWIQQVDQSWRKERVLNVPLCKEDCEQWWEDCRTSYTCKSNWHKGWNWTSGFNKCAVGAACQPFHFYFPTPTVLCNEIWTHSYKVSNYSRGSGRCIQMWFDPAQGNPNEEVARFYAAAMSGAGPWAAWPFLLSLALMLLWLLS

SEQ ID NO: 14 - protein, 895 aa, synthetic construct
  REGION 1..895: note = A synthetic FMC63-T2A-FKBP3SGFR
MALPVTALLLPLALLLHAARPEQKLISEEDLDIQMTQTTSSLSASLGDRVTISCRASQDISKYLNWYQQKPDGTVKLLIYHTSRLHSGVPSRFSGSGSGTDYSLTISNLEQEDIATYFCQQGNTLPYTFGGGTKLEITGGGGSGGGGSGGGGSEVKLQESGPGLVAPSQSLSVTCTVSGVSLPDYGVSWIRQPPRKGLEWLGVIWGSETTYYNSALKSRLTIIKDNSKSQVFLKMNSLQTDDTAIYYCAKHYYYGGSYAMDYWGQGTSVTVSSAAAIEVMYPPPYLDNEKSNGTIIHVKGKHLCPSPLFPGPSKPFWVLVVVGGVLACYSLLVTVAFIIFWVRSKRSRLLHSDYMNMTPRRPGPTRKHYQPYAPPRDFAAYRSRVKFSRSADAPAYQQGQNQLYNELNLGRREEYDVLDKRRGRDPEMGGKPRRKNPQEGLYNELQKDKMAEAYSEIGMKGERRRGKGHDGLYQGLSTATKDTYDALHMQALPPRGSGEGRGSLLTCGDVEENPGPMAQRMTTQLLLLLVWVAVVGEAQTGVQVETISPGDGRTFPKRGQTCVVHYTGMLEDGKKFDSSRDRNKPFKFMLGKQEVIRGWEEGVAQMSVGQRAKLTISPDYAYGATGHPGIIPPHATLVFDVELLKLEGGGGSGGGGSGGGGSRIAWARTELLNVCMNAKHHKEKPGPEDKLHEQCRPWRKNACCSTNTSQEAHKDVSYLYRFNWNHCGEMAPACKRHFIQDTCLYECSPNLGPWIQQVDQSWRKERVLNVPLCKEDCEQWWEDCRTSYTCKSNWHKGWNWTSGFNKCAVGAACQPFHFYFPTPTVLCNEIWTHSYKVSNYSRGSGRCIQMWFDPAQGNPNEEVARFYAAAMSGAGPWAAWPFLLSLALMLLWLLS

SEQ ID NO: 15 - protein, 1029 aa, synthetic construct
  REGION 1..1029: note = A synthetic FMC63-T2A-4M5.3SGFR
MALPVTALLLPLALLLHAARPEQKLISEEDLDIQMTQTTSSLSASLGDRVTISCRASQDISKYLNWYQQKPDGTVKLLIYHTSRLHSGVPSRFSGSGSGTDYSLTISNLEQEDIATYFCQQGNTLPYTFGGGTKLEITGGGGSGGGGSGGGGSEVKLQESGPGLVAPSQSLSVTCTVSGVSLPDYGVSWIRQPPRKGLEWLGVIWGSETTYYNSALKSRLTIIKDNSKSQVFLKMNSLQTDDTAIYYCAKHYYYGGSYAMDYWGQGTSVTVSSAAAIEVMYPPPYLDNEKSNGTIIHVKGKHLCPSPLFPGPSKPFWVLVVVGGVLACYSLLVTVAFIIFWVRSKRSRLLHSDYMNMTPRRPGPTRKHYQPYAPPRDFAAYRSRVKFSRSADAPAYQQGQNQLYNELNLGRREEYDVLDKRRGRDPEMGGKPRRKNPQEGLYNELQKDKMAEAYSEIGMKGERRRGKGHDGLYQGLSTATKDTYDALHMQALPPRGSGEGRGSLLTCGDVEENPGPMALPVTALLLPLALLLHAARPDVVMTQTPLSLPVSLGDQASISCRSSQSLVHSNGNTYLRWYLQKPGQSPKVLIYKVSNRVSGVPDRFSGSGSGTDFTLKINRVEAEDLGVYFCSQSTHVPWTFGGGTKLEIKSSADDAKKDAAKKDDAKKDDAKKDGGVKLDETGGGLVQPGGAMKLSCVTSGFTFGHYWMNWVRQSPEKGLEWVAQFRNKPYNYETYYSDSVKGRFTISRDDSKSSVYLQMNNLRVEDTGIYYCTGASYGMEYLGQGTSVTVSSGGGSRIAWARTELLNVCMNAKHHKEKPGPEDKLHEQCRPWRKNACCSTNTSQEAHKDVSYLYRFNWNHCGEMAPACKRHFIQDTCLYECSPNLGPWIQQVDQSWRKERVLNVPLCKEDCEQWWEDCRTSYTCKSNWHKGWNWTSGFNKCAVGAACQPFHFYFPTPTVLCNEIWTHSYKVSNYSRGSGRCIQMWFDPAQGNPNEEVARFYAAAMSGAGPWAAWPFLLSLALMLLWLLS

SEQ ID NO: 16 - protein, 255 aa, synthetic construct
  REGION 1..255: note = A synthetic FRb with signal peptide
MVWKWMPLLLLLVCVATMCSAQDRTDLLNVCMDAKHHKTKPGPEDKLHDQCSPWKKNACCTASTSQELHKDTSRLYNFNWDHCGKMEPACKRHFIQDTCLYECSPNLGPWIQQVNQSWRKERFLDVPLCKEDCQRWWEDCHTSHTCKSNWHRGWDWTSGVNKCPAGALCRTFESYFPTPAALCEGLWSHSYKVSNYSRGSGRCIQMWFDSAQGNPNEEVARFYAAAMHVNAGEMLHGTGGLLLSLALMLQLWLLG

SEQ ID NO: 17 - protein, 335 aa, synthetic construct
  REGION 1..335: note = A synthetic uPAR with signal peptide
MGHPPLLPLLLLLHTCVPASWGLRCMQCKTNGDCRVEECALGQDLCRTTIVRLWEEGEELELVEKSCTHSEKTNRTLSYRTGLKITSLTEVVCGLDLCNQGNSGRAVTYSRSRYLECISCGSSDMSCERGRHQSLQCRSPEEQCLDVVTHWIQEGEEGRPKDDRHLRGCGYLPGCPGSNGFHNNDTFHFLKCCNTTKCNEGPILELENLPQNGRQCYSCKGNSTHGCSSEETFLIDCRGPMNQCLVATGTHEPKNQSYMVRGCATASMCQHAHLGDAFSMNHIDVSCCTKSGCNHPDLDVQYRSGAAPQPGPAHLSLTITLLMTARLWGGTLLWT

SEQ ID NO: 18 - protein, 187 aa, synthetic construct
  REGION 1..187: note = A synthetic DHFR
MVGSLNCIVAVSQNMGIGKNGDLPWPPLRNEFRYFQRMTTTSSVEGKQNLVIMGKKTWFSIPEKNRPLKGRINLVLSRELKEPPQGAHFLSRSLDDALKLTEQPELANKVDMVWIVGGSSVYKEAMNHPGHLKLFVTRIMQDFESDTFFPEIDLEKYKLLPEYPGVLSDVQEEKGIKYKFEVYEKND

SEQ ID NO: 19 - protein, 255 aa, synthetic construct
  REGION 1..255: note = A synthetic scFv against FITC: 4M5.3(Kd = 200pM)
DVVMTQTPLSLPVSLGDQASISCRSSQSLVHSNGNTYLRWYLQKPGQSPKVLIYKVSNRVSGVPDRFSGSGSGTDFTLKINRVEAEDLGVYFCSQSTHVPWTFGGGTKLEIKSSADDAKKDAAKKDDAKKDDAKKDGGVKLDETGGGLVQPGGAMKLSCVTSGFTFGHYWMNWVRQSPEKGLEWVAQFRNKPYNYETYYSDSVKGRFTISRDDSKSSVYLQMNNLRVEDTGIYYCTGASYGMEYLGQGTSVTVSS

SEQ ID NO: 20 - protein, 244 aa, synthetic construct
  REGION 1..244: note = A synthetic scFv against FITC 4D5Flu (Kd=10nM)
DIQMTQSPSSLSASVGDRVTITCRASQDVNTAVAWYQQKPGKAPKLLIYSASFLYSGVPSRFSGSRSGTDFTLTISSLQPEDFATYYCQQHYTTPPTFGQGTKVEIKRTGGGGSGGGGSGGGGSEVQLVESGGGLVQPGGSLRLSCAASGFNIKDTYIHWVRQAPGKGLEWVARIYPTNGYTRYADSVKGRFTISADTSKNTAYLQMNSLRAEDTAVYYCSRWGGDGFYAMDYWGQGTLVTVSS

SEQ ID NO: 21 - protein, 244 aa, synthetic construct
  REGION 1..244: note = A synthetic scFv against DNP SPE7
QAVVTQESALTTSPGETVTLTCRSSTGAVTTSNYANWVQEKPDHLFTGLIGGTNNRAPGVPARFSGSLIGDKAALTITGAQTEDEAIYFCALWYSNHLVFGGGTKLTVLGGGGSGGGGSGGGGSEVQLQQPGAELVKPGASVKLSCKASGYTFTSYWMHWVKQRPGRGLEWIGRIDPNGGGTKYNEKFKSKATLTVDKPSSTAYMQLSSLTSEDSAVYYCARMWYYGTYYFDYWGQGTTLTVSS

SEQ ID NO: 22 - protein, 4 aa, synthetic construct
  REGION 1..4: note = A synthetic sequence
DDRD